European Patent Specification EP 3 784 695 B1, published August 9, 2023. Title: USE OF LENTIVECTOR-TRANSDUCED T-RAPA CELLS FOR AMELIORATION OF LYSOSOMAL STORAGE DISORDERS. Applicant: THE MEDICAL COLLEGE OF WISCONSIN, INC. Medin, Jeffrey Fowler, Daniel Nagree, Murtaza Felizardo, Tania. The sequence listing filed with the application follows.

SEQUENCE LISTING (11 sequences)

SEQ ID NO: 1 - DNA, 1290 bp, Artificial Sequence
  AGA transgene
atgcaacttcgaaacccagagctccacctcggatgtgcccttgctctgaggttcctggcgctggtgtcttgggatatacccggagcacgcgctctggacaacgggctggcccggactccaaccatgggttggctccattgggaaaggtttatgtgcaacttggactgccaggaagaacccgactcctgtatttccgagaaactcttcatggagatggccgagctgatggttagcgaaggctggaaggatgccggttatgaatacttgtgtatcgacgattgttggatggctccccagcgggacagtgaaggacgactccaggcagatccgcaacggttccctcatggcatacggcagctcgccaattacgtgcacagcaagggtttgaagctggggatatatgctgacgtgggcaacaaaacctgtgctggtttccccggcagcttcggctactatgatatagatgcacaaaccttcgctgattggggcgtggacctgcttaaatttgacggctgttactgcgacagcttggaaaacctcgccgatggatataaacacatgagccttgcactcaatcggactggccggagcattgtctactcttgcgagtggccattgtacatgtggcctttccagaagcctaactatacggagattagacagtattgtaatcactggagaaactttgcagatatcgacgactcatggaagtccatcaaatctattctggactggacttcattcaatcaggagcgcatcgtcgatgttgccggtccaggtggatggaacgaccctgacatgctcgtaattgggaatttcggactgtcctggaatcagcaggtcacacagatggctttgtgggctatcatggcagccccactctttatgtctaacgatttgcggcatatttcaccacaggccaaagccctgctgcaagataaggacgtcatagcgattaaccaggacccactgggaaagcagggctaccagctgagacagggcgacaattttgaggtctgggaaagacctcttagcgggctggcgtgggccgtagccatgattaatcgccaggaaattggcggccctcgctcttacactatcgcggtcgccagtctgggcaagggagtcgcttgtaaccccgcctgcttcataactcagttgctgcccgtgaaacggaagctgggcttctatgaatggactagcagactccgcagtcatattaatccgactggtacggtgctgctgcaactggagaataccatgcagatgtcacttaaggatcttctgtga

SEQ ID NO: 2 - DNA, 8767 bp, Artificial Sequence
  Lentiviral vector comprising AGA transgene
aaattgtaagcgttaatattttgttaaaattcgcgttaaatttttgttaaatcagctcattttttaaccaataggccgaaatcggcaaaatcccttataaatcaaaagaatagaccgagatagggttgagtgttgttccagtttggaacaagagtccactattaaagaacgtggactccaacgtcaaagggcgaaaaaccgtctatcagggcgatggcccactacgtgaaccatcaccctaatcaagttttttggggtcgaggtgccgtaaagcactaaatcggaaccctaaagggagcccccgatttagagcttgacggggaaagccggcgaacgtggcgagaaaggaagggaagaaagcgaaaggagcgggcgctagggcgctggcaagtgtagcggtcacgctgcgcgtaaccaccacacccgccgcgcttaatgcgccgctacagggcgcgtccattcgccattcaggctgcgcaactgttgggaagggcgatcggtgcgggcctcttcgctattacgccagctggcgaaagggggatgtgctgcaaggcgattaagttgggtaacgccagggttttcccagtcacgacgttgtaaaacgacggccagtgaattgtaatacgactcactatagggcgaattgggcccgacgtcgcatgcttggaagggctaattcactcccaaagaagacaagatatccttgatctgtggatctaccacacacaaggctacttccctgattagcagaactacacaccagggccaggggtcagatatccactgacctttggatggtgctacaagctagtaccagttgagccagataaggtagaagaggccaataaaggagagaacaccagcttgttacaccctgtgagcctgcatgggatggatgacccggagagagaagtgttagagtggaggtttgacagccgcctagcatttcatcacgtggcccgagagctgcatccggagtacttcaagaactgctgatatcgagcttgctacaagggactttccgctggggactttccagggaggcgtggcctgggcgggactggggagtggcgagccctcagatcctgcatataagcagctgctttttgcctgtactgggtctctctggttagaccagatctgagcctgggagctctctggctaactagggaacccactgcttaagcctcaataaagcttgccttgagtgcttcaagtagtgtgtgcccgtctgttgtgtgactctggtaactagagatccctcagacccttttagtcagtgtggaaaatctctagcagtggcgcccgaacagggacttgaaagcgaaagggaaaccagaggagctctctcgacgcaggactcggcttgctgaagcgcgcacggcaagaggcgaggggcggcgactggtgagtacgccaaaaattttgactagcggaggctagaaggagagagatgggtgcgagagcgtcagtattaagcgggggagaattagatcgcgatgggaaaaaattcggttaaggccagggggaaagaaaaaatataaattaaaacatatagtatgggcaagcagggagctagaacgattcgcagttaatcctggcctgttagaaacatcagaaggctgtagacaaatactgggacagctacaaccatcccttcagacaggatcagaagaacttagatcattatataatacagtagcaaccctctattgtgtgcatcaaaggatagagataaaagacaccaaggaagctttagacaagatagaggaagagcaaaacaaaagtaagaccaccgcacagcaagcggccgctgatcttcagacctggaggaggagatatgagggacaattggagaagtgaattatataaatataaagtagtaaaaattgaaccattaggagtagcacccaccaaggcaaagagaagagtggtgcagagagaaaaaagagcagtgggaataggagctttgttccttgggttcttgggagcagcaggaagcactatgggcgcagcgtcaatgacgctgacggtacaggccagacaattattgtctggtatagtgcagcagcagaacaatttgctgagggctattgaggcgcaacagcatctgttgcaactcacagtctggggcatcaagcagctccaggcaagaatcctggctgtggaaagatacctaaaggatcaacagctcctggggatttggggttgctctggaaaactcatttgcaccactgctgtgccttggaatgctagttggagtaataaatctctggaacagatttggaatcacacgacctggatggagtgggacagagaaattaacaattacacaagcttaatacactccttaattgaagaatcgcaaaaccagcaagaaaagaatgaacaagaattattggaattagataaatgggcaagtttgtggaattggtttaacataacaaattggctgtggtatataaaattattcataatgatagtaggaggcttggtaggtttaagaatagtttttgctgtactttctatagtgaatagagttaggcagggatattcaccattatcgtttcagacccacctcccaaccccgaggggacccgacaggcccgaaggaatagaagaagaaggtggagagagagacagagacagatccattcgattagtgaacggatctcgacgggatcgattttaaaagaaaaggggggattggggggtacagtgcaggggaaagaatagtagacataatagcaacagacatacaaactaaagaattacaaaaacaaattacaaaaattcaaaattttatcgataagctttgcaaagatggataaagttttaaacagagaggaatctttgcagctaatggaccttctaggtcttgaaaggagtgggaattggctccggtgcccgtcagtgggcagagcgcacatcgcccacagtccccgagaagttggggggaggggtcggcaattgaaccggtgcctagagaaggtggcgcggggtaaactgggaaagtgatgtcgtgtactggctccgcctttttcccgagggtgggggagaaccgtatataagtgcagtagtcgccgtgaacgttctttttcgcaacgggtttgccgccagaacacaggtaagtgccgtgtgtggttcccgcgggcctggcctctttacgggttatggcccttgcgtgccttgaattacttccacctggctgcagtacgtgattcttgatcccgagcttcgggttggaagtgggtgggagagttcgaggccttgcgcttaaggagccccttcgcctcgtgcttgagttgaggcctggcctgggcgctggggccgccgcgtgcgaatctggtggcaccttcgcgcctgtctcgctgctttcgataagtctctagccatttaaaatttttgatgacctgctgcgacgctttttttctggcaagatagtcttgtaaatgcgggccaagatctgcacactggtatttcggtttttggggccgcgggcggcgacggggcccgtgcgtcccagcgcacatgttcggcgaggcggggcctgcgagcgcggccaccgagaatcggacgggggtagtctcaagctggccggcctgctctggtgcctggcctcgcgccgccgtgtatcgccccgccctgggcggcaaggctggcccggtcggcaccagttgcgtgagcggaaagatggccgcttcccggccctgctgcagggagctcaaaatggaggacgcggcgctcgggagagcgggcgggtgagtcacccacacaaaggaaaagggcctttccgtcctcagccgtcgcttcatgtgactccacggagtaccgggcgccgtccaggcacctcgattagttctcgagcttttggagtacgtcgtctttaggttggggggaggggttttatgcgatggagtttccccacactgagtgggtggagactgaagttaggccagcttggcacttgatgtaattctccttggaatttgccctttttgagtttggatcttggttcattctcaagcctcagacagtggttcaaagtttttttcttccatttcaggtgtcgtgaggaattcgccaccatgcaacttcgaaacccagagctccacctcggatgtgcccttgctctgaggttcctggcgctggtgtcttgggatatacccggagcacgcgctctggacaacgggctggcccggactccaaccatgggttggctccattgggaaaggtttatgtgcaacttggactgccaggaagaacccgactcctgtatttccgagaaactcttcatggagatggccgagctgatggttagcgaaggctggaaggatgccggttatgaatacttgtgtatcgacgattgttggatggctccccagcgggacagtgaaggacgactccaggcagatccgcaacggttccctcatggcatacggcagctcgccaattacgtgcacagcaagggtttgaagctggggatatatgctgacgtgggcaacaaaacctgtgctggtttccccggcagcttcggctactatgatatagatgcacaaaccttcgctgattggggcgtggacctgcttaaatttgacggctgttactgcgacagcttggaaaacctcgccgatggatataaacacatgagccttgcactcaatcggactggccggagcattgtctactcttgcgagtggccattgtacatgtggcctttccagaagcctaactatacggagattagacagtattgtaatcactggagaaactttgcagatatcgacgactcatggaagtccatcaaatctattctggactggacttcattcaatcaggagcgcatcgtcgatgttgccggtccaggtggatggaacgaccctgacatgctcgtaattgggaatttcggactgtcctggaatcagcaggtcacacagatggctttgtgggctatcatggcagccccactctttatgtctaacgatttgcggcatatttcaccacaggccaaagccctgctgcaagataaggacgtcatagcgattaaccaggacccactgggaaagcagggctaccagctgagacagggcgacaattttgaggtctgggaaagacctcttagcgggctggcgtgggccgtagccatgattaatcgccaggaaattggcggccctcgctcttacactatcgcggtcgccagtctgggcaagggagtcgcttgtaaccccgcctgcttcataactcagttgctgcccgtgaaacggaagctgggcttctatgaatggactagcagactccgcagtcatattaatccgactggtacggtgctgctgcaactggagaataccatgcagatgtcacttaaggatcttctgtgagaacccgggatccaagcttcaattgtggtcactcgacaatcaacctctggattacaaaatttgtgaaagattgactggtattcttaactatgttgctccttttacgctatgtggatacgctgctttaatgcctttgtatcatgctattgcttcccgtatggctttcattttctcctccttgtataaatcctggttgctgtctctttatgaggagttgtggcccgttgtcaggcaacgtggcgtggtgtgcactgtgtttgctgacgcaacccccactggttggggcattgccaccacctgtcagctcctttccgggactttcgctttccccctccctattgccacggcggaactcatcgccgcctgccttgcccgctgctggacaggggctcggctgttgggcactgacaattccgtggtgttgtcggggaagctgacgtcctttccatggctgctcgcctgtgttgccacctggattctgcgcgggacgtccttctgctacgtcccttcggccctcaatccagcggaccttccttcccgcggcctgctgccggctctgcggcctcttccgcgtcttcgccttcgccctcagacgagtcggatctccctttgggccgcctccccgcctgctcgagacctagaaaaacatggagcaatcacaagtagcaatacagcagctaccaatgctgattgtgcctggctagaagcacaagaggaggaggaggtgggttttccagtcacacctcaggtacctttaagaccaatgacttacaaggcagctgtagatcttagccactttttaaaagaaaaggggggactggaagggctaattcactcccaacgaagacaagatctgctttttgcttgtactgggtctctctggttagaccagatctgagcctgggagctctctggctaactagggaacccactgcttaagcctcaataaagcttgccttgagtgcttcaagtagtgtgtgcccgtctgttgtgtgactctggtaactagagatccctcagacccttttagtcagtgtggaaaatctctagcagtagtagttcatgtcatcttattattcagtatttataacttgcaaagaaatgaatatcagagagtgagaggacgcgttggatgcatagcttgagtattctatagtgtcacctaaatagcttggcgtaatcatggtcatagctgtttcctgtgtgaaattgttatccgctcacaattccacacaacatacgagccggaagcataaagtgtaaagcctggggtgcctaatgagtgagctaactcacattaattgcgttgcgctcactgcccgctttccagtcgggaaacctgtcgtgccagctgcattaatgaatcggccaacgcgcggggagaggcggtttgcgtattgggcgctcttccgcttcctcgctcactgactcgctgcgctcggtcgttcggctgcggcgagcggtatcagctcactcaaaggcggtaatacggttatccacagaatcaggggataacgcaggaaagaacatgtgagcaaaaggccagcaaaaggccaggaaccgtaaaaaggccgcgttgctggcgtttttccataggctccgcccccctgacgagcatcacaaaaatcgacgctcaagtcagaggtggcgaaacccgacaggactataaagataccaggcgtttccccctggaagctccctcgtgcgctctcctgttccgaccctgccgcttaccggatacctgtccgcctttctcccttcgggaagcgtggcgctttctcatagctcacgctgtaggtatctcagttcggtgtaggtcgttcgctccaagctgggctgtgtgcacgaaccccccgttcagcccgaccgctgcgccttatccggtaactatcgtcttgagtccaacccggtaagacacgacttatcgccactggcagcagccactggtaacaggattagcagagcgaggtatgtaggcggtgctacagagttcttgaagtggtggcctaactacggctacactagaagaacagtatttggtatctgcgctctgctgaagccagttaccttcggaaaaagagttggtagctcttgatccggcaaacaaaccaccgctggtagcggtggtttttttgtttgcaagcagcagattacgcgcagaaaaaaaggatctcaagaagatcctttgatcttttctacggggtctgacgctcagtggaacgaaaactcacgttaagggattttggtcatgagattatcaaaaaggatcttcacctagatccttttaaattaaaaatgaagttttaaatcaatctaaagtatatatgagtaaacttggtctgacagttaccaatgcttaatcagtgaggcacctatctcagcgatctgtctatttcgttcatccatagttgcctgactccccgtcgtgtagataactacgatacgggagggcttaccatctggccccagtgctgcaatgataccgcgagacccacgctcaccggctccagatttatcagcaataaaccagccagccggaagggccgagcgcagaagtggtcctgcaactttatccgcctccatccagtctattaattgttgccgggaagctagagtaagtagttcgccagttaatagtttgcgcaacgttgttgccattgctacaggcatcgtggtgtcacgctcgtcgtttggtatggcttcattcagctccggttcccaacgatcaaggcgagttacatgatcccccatgttgtgcaaaaaagcggttagctccttcggtcctccgatcgttgtcagaagtaagttggccgcagtgttatcactcatggttatggcagcactgcataattctcttactgtcatgccatccgtaagatgcttttctgtgactggtgagtactcaaccaagtcattctgagaatagtgtatgcggcgaccgagttgctcttgcccggcgtcaatacgggataataccgcgccacatagcagaactttaaaagtgctcatcattggaaaacgttcttcggggcgaaaactctcaaggatcttaccgctgttgagatccagttcgatgtaacccactcgtgcacccaactgatcttcagcatcttttactttcaccagcgtttctgggtgagcaaaaacaggaaggcaaaatgccgcaaaaaagggaataagggcgacacggaaatgttgaatactcatactcttcctttttcaatattattgaagcatttatcagggttattgtctcatgagcggatacatatttgaatgtatttagaaaaataaacaaataggggttccgcgcacatttccccgaaaagtgccacctgatgcggtgtgaaataccgcacagatgcgtaaggagaaaataccgcatcagg

SEQ ID NO: 3 - DNA, 11298 bp, Artificial Sequence
  Dual promoter lentiviral vector comprising AGA transgene
aaattgtaagcgttaatattttgttaaaattcgcgttaaatttttgttaaatcagctcattttttaaccaataggccgaaatcggcaaaatcccttataaatcaaaagaatagaccgagatagggttgagtgttgttccagtttggaacaagagtccactattaaagaacgtggactccaacgtcaaagggcgaaaaaccgtctatcagggcgatggcccactacgtgaaccatcaccctaatcaagttttttggggtcgaggtgccgtaaagcactaaatcggaaccctaaagggagcccccgatttagagcttgacggggaaagccggcgaacgtggcgagaaaggaagggaagaaagcgaaaggagcgggcgctagggcgctggcaagtgtagcggtcacgctgcgcgtaaccaccacacccgccgcgcttaatgcgccgctacagggcgcgtccattcgccattcaggctgcgcaactgttgggaagggcgatcggtgcgggcctcttcgctattacgccagctggcgaaagggggatgtgctgcaaggcgattaagttgggtaacgccagggttttcccagtcacgacgttgtaaaacgacggccagtgaattgtaatacgactcactatagggcgaattgggcccgacgtcgcatgcttggaagggctaattcactcccaaagaagacaagatatccttgatctgtggatctaccacacacaaggctacttccctgattagcagaactacacaccagggccaggggtcagatatccactgacctttggatggtgctacaagctagtaccagttgagccagataaggtagaagaggccaataaaggagagaacaccagcttgttacaccctgtgagcctgcatgggatggatgacccggagagagaagtgttagagtggaggtttgacagccgcctagcatttcatcacgtggcccgagagctgcatccggagtacttcaagaactgctgatatcgagcttgctacaagggactttccgctggggactttccagggaggcgtggcctgggcgggactggggagtggcgagccctcagatcctgcatataagcagctgctttttgcctgtactgggtctctctggttagaccagatctgagcctgggagctctctggctaactagggaacccactgcttaagcctcaataaagcttgccttgagtgcttcaagtagtgtgtgcccgtctgttgtgtgactctggtaactagagatccctcagacccttttagtcagtgtggaaaatctctagcagtggcgcccgaacagggacttgaaagcgaaagggaaaccagaggagctctctcgacgcaggactcggcttgctgaagcgcgcacggcaagaggcgaggggcggcgactggtgagtacgccaaaaattttgactagcggaggctagaaggagagagatgggtgcgagagcgtcagtattaagcgggggagaattagatcgcgatgggaaaaaattcggttaaggccagggggaaagaaaaaatataaattaaaacatatagtatgggcaagcagggagctagaacgattcgcagttaatcctggcctgttagaaacatcagaaggctgtagacaaatactgggacagctacaaccatcccttcagacaggatcagaagaacttagatcattatataatacagtagcaaccctctattgtgtgcatcaaaggatagagataaaagacaccaaggaagctttagacaagatagaggaagagcaaaacaaaagtaagaccaccgcacagcaagcggccgctgatcttcagacctggaggaggagatatgagggacaattggagaagtgaattatataaatataaagtagtaaaaattgaaccattaggagtagcacccaccaaggcaaagagaagagtggtgcagagagaaaaaagagcagtgggaataggagctttgttccttgggttcttgggagcagcaggaagcactatgggcgcagcgtcaatgacgctgacggtacaggccagacaattattgtctggtatagtgcagcagcagaacaatttgctgagggctattgaggcgcaacagcatctgttgcaactcacagtctggggcatcaagcagctccaggcaagaatcctggctgtggaaagatacctaaaggatcaacagctcctggggatttggggttgctctggaaaactcatttgcaccactgctgtgccttggaatgctagttggagtaataaatctctggaacagatttggaatcacacgacctggatggagtgggacagagaaattaacaattacacaagcttaatacactccttaattgaagaatcgcaaaaccagcaagaaaagaatgaacaagaattattggaattagataaatgggcaagtttgtggaattggtttaacataacaaattggctgtggtatataaaattattcataatgatagtaggaggcttggtaggtttaagaatagtttttgctgtactttctatagtgaatagagttaggcagggatattcaccattatcgtttcagacccacctcccaaccccgaggggacccgacaggcccgaaggaatagaagaagaaggtggagagagagacagagacagatccattcgattagtgaacggatctcgacgggatcgattttaaaagaaaaggggggattggggggtacagtgcaggggaaagaatagtagacataatagcaacagacatacaaactaaagaattacaaaaacaaattacaaaaattcaaaattttatcgataagctttgcaaagatggataaagttttaaacagagaggaatctttgcagctaatggaccttctaggtctgaccccgtacgcctcgagagatctgatcataatcagccataccacatttgtagaggttttacttgctttaaaaaacctcccacacctccccctgaacctgaaacataaaatgaatgcaattgttgttgttaacttgtttattgcagcttataatggttacaaataaggcaatagcatcacaaatttcacaaataaggcatttttttcactgcattctagttttggtttgtccaaactcatcaatgtatcttatcatgtctggatctcaaatccctcggaagctgcgcctgtcttaggttggagtgatacatttttatcacttttacccgtctttggattaggcagtagctctgacggccctcctgtcttaggttagtgaaaaatgtcactctcttacccgtcattggctgtccagcttagctcgcaggggaggtggtctgcctgcaggttagaacagtctcttttcgtatgagtgcagtgagtggacgccgccttcgacctgggctgaagaagttcttttctcgaacttcagttcgccggaatacatcattgcccgcacctgtgtcaggctcttagcgccgatatcctggcatgaatgctgaattccggcgatcaggtaaggcacgaatttgtgaatactgcccttatcctggacagctccagacacgccctgtgcgactttgatcttgtctgcctcggaaaaatacctgttctgagaggacagatgcttatccatggcgtccagtgaccccatgcccctatatttcttcagtctgaacccatcactaaagaagtactcgccgggggcttctgtggttgcagccagcaggctgcccatcatcactgtgcttgcccccagagccagggcttttgcgatgtggcccacattctgaattcccccgtcagcgatcactgggactccgaatctccgggcatactcgtacaccttgtagacagcagttgcctgaggtcgtccacaggccagcacttcctgaatgatgcagattgatccactccccattccgaccctcagagcatccactcctgcgtcaatcaggtttttggcctgggctgcggtcacgacattgcctccgatgacctgcagatttgggtacttgtccttaatgtacttgatcatattaatctggaagatgctgtttccctggcttgaatccagcacgaccacgtccacccctgcctgagccagcagatccaggcgatatttatcgtcctcgtgtgtgccaatagcggctccacacagcagctgtttctttgcgtccttactagccagagggtaatctcgatttttcttcaggtcggtgcgggcaatgattgccaccagctcatcgtcttcattcacgataggcagttttcctttcttagaccgctgcagaatctcgttggcttccttcagtgtgatgccggcaggtgcgaccaccagatcttcgcgtttggtcataatctcttccagaaaacagtcatgctcttcctccttcaggaaatcgatgtctcgactagaaatgattcccaccagtcggctgcccattcgtccagtatctgtaatggggatgccgcaaaatccgtgcctagctttggcctcgaacacatcgcggaccctgtccttggggctcaggaccactgggtcggtgataaagccctgttcgtatttcttcacctttctgacctcattggcctgaaattctggagtgcagttatggtgaatgaacccgatcccgcctgtcagtgccatagcaatggccatgccagcctcggtgacagtgtccataggggagctcaccaggggtgtcttcagggtgattttcttggtcagggcagaagtcagatccacctggtctgcggtaaaatcaatatagccgggcaggatcaggaagtcgttgtaagtcagcccgtctccacaattaaacagctgctgggcggtcagtccatcatcagggacataggaagtgcctccagaaatcaggtagtcggccatggtggcgctagccctggggagagaggtcggtgattcggtcaacgagggagccgactgccgacgtgcgctccggaggcttgcagaatgcggaacaccgcgcgggcaggaacagggcccacactaccgccccacaccccgcctcccgcaccgccccttcccggccgctgctctcggcgcgccccgctgagcagccgctattggccacagcccatcgcggtcggcgcgctgccattgctccctggcgctgtccgtctgcgagggtactagtgagacgtgcggcttccgtttgtcacgtccggcacgccgcgaaccgcaaggaaccttcccgacttaggggcggagcaggaagcgtcgccggggggcccacaagggtagcggcgaagatccgggtgacgctgcgaacggacgtgaagaatgtgcgagacccagggtcggcgccgctgcgtttcccggaaccacgcccagagcagccgcgtccctgcgcaaacccagggctgccaaggaaaaggcgcaaccccaaccccgtggttaattaaggtgaaaggagtgggaattggctccggtgcccgtcagtgggcagagcgcacatcgcccacagtccccgagaagttggggggaggggtcggcaattgaaccggtgcctagagaaggtggcgcggggtaaactgggaaagtgatgtcgtgtactggctccgcctttttcccgagggtgggggagaaccgtatataagtgcagtagtcgccgtgaacgttctttttcgcaacgggtttgccgccagaacacaggtaagtgccgtgtgtggttcccgcgggcctggcctctttacgggttatggcccttgcgtgccttgaattacttccacctggctgcagtacgtgattcttgatcccgagcttcgggttggaagtgggtgggagagttcgaggccttgcgcttaaggagccccttcgcctcgtgcttgagttgaggcctggcctgggcgctggggccgccgcgtgcgaatctggtggcaccttcgcgcctgtctcgctgctttcgataagtctctagccatttaaaatttttgatgacctgctgcgacgctttttttctggcaagatagtcttgtaaatgcgggccaagatctgcacactggtatttcggtttttggggccgcgggcggcgacggggcccgtgcgtcccagcgcacatgttcggcgaggcggggcctgcgagcgcggccaccgagaatcggacgggggtagtctcaagctggccggcctgctctggtgcctggcctcgcgccgccgtgtatcgccccgccctgggcggcaaggctggcccggtcggcaccagttgcgtgagcggaaagatggccgcttcccggccctgctgcagggagctcaaaatggaggacgcggcgctcgggagagcgggcgggtgagtcacccacacaaaggaaaagggcctttccgtcctcagccgtcgcttcatgtgactccacggagtaccgggcgccgtccaggcacctcgattagttctcgagcttttggagtacgtcgtctttaggttggggggaggggttttatgcgatggagtttccccacactgagtgggtggagactgaagttaggccagcttggcacttgatgtaattctccttggaatttgccctttttgagtttggatcttggttcattctcaagcctcagacagtggttcaaagtttttttcttccatttcaggtgtcgtgaggaattcgccaccatgcaacttcgaaacccagagctccacctcggatgtgcccttgctctgaggttcctggcgctggtgtcttgggatatacccggagcacgcgctctggacaacgggctggcccggactccaaccatgggttggctccattgggaaaggtttatgtgcaacttggactgccaggaagaacccgactcctgtatttccgagaaactcttcatggagatggccgagctgatggttagcgaaggctggaaggatgccggttatgaatacttgtgtatcgacgattgttggatggctccccagcgggacagtgaaggacgactccaggcagatccgcaacggttccctcatggcatacggcagctcgccaattacgtgcacagcaagggtttgaagctggggatatatgctgacgtgggcaacaaaacctgtgctggtttccccggcagcttcggctactatgatatagatgcacaaaccttcgctgattggggcgtggacctgcttaaatttgacggctgttactgcgacagcttggaaaacctcgccgatggatataaacacatgagccttgcactcaatcggactggccggagcattgtctactcttgcgagtggccattgtacatgtggcctttccagaagcctaactatacggagattagacagtattgtaatcactggagaaactttgcagatatcgacgactcatggaagtccatcaaatctattctggactggacttcattcaatcaggagcgcatcgtcgatgttgccggtccaggtggatggaacgaccctgacatgctcgtaattgggaatttcggactgtcctggaatcagcaggtcacacagatggctttgtgggctatcatggcagccccactctttatgtctaacgatttgcggcatatttcaccacaggccaaagccctgctgcaagataaggacgtcatagcgattaaccaggacccactgggaaagcagggctaccagctgagacagggcgacaattttgaggtctgggaaagacctcttagcgggctggcgtgggccgtagccatgattaatcgccaggaaattggcggccctcgctcttacactatcgcggtcgccagtctgggcaagggagtcgcttgtaaccccgcctgcttcataactcagttgctgcccgtgaaacggaagctgggcttctatgaatggactagcagactccgcagtcatattaatccgactggtacggtgctgctgcaactggagaataccatgcagatgtcacttaaggatcttctgtgagaacccgggatccaagcttcaattgtggtcactcgacaatcaacctctggattacaaaatttgtgaaagattgactggtattcttaactatgttgctccttttacgctatgtggatacgctgctttaatgcctttgtatcatgctattgcttcccgtatggctttcattttctcctccttgtataaatcctggttgctgtctctttatgaggagttgtggcccgttgtcaggcaacgtggcgtggtgtgcactgtgtttgctgacgcaacccccactggttggggcattgccaccacctgtcagctcctttccgggactttcgctttccccctccctattgccacggcggaactcatcgccgcctgccttgcccgctgctggacaggggctcggctgttgggcactgacaattccgtggtgttgtcggggaagctgacgtcctttccatggctgctcgcctgtgttgccacctggattctgcgcgggacgtccttctgctacgtcccttcggccctcaatccagcggaccttccttcccgcggcctgctgccggctctgcggcctcttccgcgtcttcgccttcgccctcagacgagtcggatctccctttgggccgcctccccgcctgctcgagacctagaaaaacatggagcaatcacaagtagcaatacagcagctaccaatgctgattgtgcctggctagaagcacaagaggaggaggaggtgggttttccagtcacacctcaggtacctttaagaccaatgacttacaaggcagctgtagatcttagccactttttaaaagaaaaggggggactggaagggctaattcactcccaacgaagacaagatctgctttttgcttgtactgggtctctctggttagaccagatctgagcctgggagctctctggctaactagggaacccactgcttaagcctcaataaagcttgccttgagtgcttcaagtagtgtgtgcccgtctgttgtgtgactctggtaactagagatccctcagacccttttagtcagtgtggaaaatctctagcagtagtagttcatgtcatcttattattcagtatttataacttgcaaagaaatgaatatcagagagtgagaggacgcgttggatgcatagcttgagtattctatagtgtcacctaaatagcttggcgtaatcatggtcatagctgtttcctgtgtgaaattgttatccgctcacaattccacacaacatacgagccggaagcataaagtgtaaagcctggggtgcctaatgagtgagctaactcacattaattgcgttgcgctcactgcccgctttccagtcgggaaacctgtcgtgccagctgcattaatgaatcggccaacgcgcggggagaggcggtttgcgtattgggcgctcttccgcttcctcgctcactgactcgctgcgctcggtcgttcggctgcggcgagcggtatcagctcactcaaaggcggtaatacggttatccacagaatcaggggataacgcaggaaagaacatgtgagcaaaaggccagcaaaaggccaggaaccgtaaaaaggccgcgttgctggcgtttttccataggctccgcccccctgacgagcatcacaaaaatcgacgctcaagtcagaggtggcgaaacccgacaggactataaagataccaggcgtttccccctggaagctccctcgtgcgctctcctgttccgaccctgccgcttaccggatacctgtccgcctttctcccttcgggaagcgtggcgctttctcatagctcacgctgtaggtatctcagttcggtgtaggtcgttcgctccaagctgggctgtgtgcacgaaccccccgttcagcccgaccgctgcgccttatccggtaactatcgtcttgagtccaacccggtaagacacgacttatcgccactggcagcagccactggtaacaggattagcagagcgaggtatgtaggcggtgctacagagttcttgaagtggtggcctaactacggctacactagaagaacagtatttggtatctgcgctctgctgaagccagttaccttcggaaaaagagttggtagctcttgatccggcaaacaaaccaccgctggtagcggtggtttttttgtttgcaagcagcagattacgcgcagaaaaaaaggatctcaagaagatcctttgatcttttctacggggtctgacgctcagtggaacgaaaactcacgttaagggattttggtcatgagattatcaaaaaggatcttcacctagatccttttaaattaaaaatgaagttttaaatcaatctaaagtatatatgagtaaacttggtctgacagttaccaatgcttaatcagtgaggcacctatctcagcgatctgtctatttcgttcatccatagttgcctgactccccgtcgtgtagataactacgatacgggagggcttaccatctggccccagtgctgcaatgataccgcgagacccacgctcaccggctccagatttatcagcaataaaccagccagccggaagggccgagcgcagaagtggtcctgcaactttatccgcctccatccagtctattaattgttgccgggaagctagagtaagtagttcgccagttaatagtttgcgcaacgttgttgccattgctacaggcatcgtggtgtcacgctcgtcgtttggtatggcttcattcagctccggttcccaacgatcaaggcgagttacatgatcccccatgttgtgcaaaaaagcggttagctccttcggtcctccgatcgttgtcagaagtaagttggccgcagtgttatcactcatggttatggcagcactgcataattctcttactgtcatgccatccgtaagatgcttttctgtgactggtgagtactcaaccaagtcattctgagaatagtgtatgcggcgaccgagttgctcttgcccggcgtcaatacgggataataccgcgccacatagcagaactttaaaagtgctcatcattggaaaacgttcttcggggcgaaaactctcaaggatcttaccgctgttgagatccagttcgatgtaacccactcgtgcacccaactgatcttcagcatcttttactttcaccagcgtttctgggtgagcaaaaacaggaaggcaaaatgccgcaaaaaagggaataagggcgacacggaaatgttgaatactcatactcttcctttttcaatattattgaagcatttatcagggttattgtctcatgagcggatacatatttgaatgtatttagaaaaataaacaaataggggttccgcgcacatttccccgaaaagtgccacctgatgcggtgtgaaataccgcacagatgcgtaaggagaaaataccgcatcagg

SEQ ID NO: 4 - DNA, 9095 bp, Artificial Sequence
  Lentiviral vector comprising GBA transgene
aaattgtaagcgttaatattttgttaaaattcgcgttaaatttttgttaaatcagctcattttttaaccaataggccgaaatcggcaaaatcccttataaatcaaaagaatagaccgagatagggttgagtgttgttccagtttggaacaagagtccactattaaagaacgtggactccaacgtcaaagggcgaaaaaccgtctatcagggcgatggcccactacgtgaaccatcaccctaatcaagttttttggggtcgaggtgccgtaaagcactaaatcggaaccctaaagggagcccccgatttagagcttgacggggaaagccggcgaacgtggcgagaaaggaagggaagaaagcgaaaggagcgggcgctagggcgctggcaagtgtagcggtcacgctgcgcgtaaccaccacacccgccgcgcttaatgcgccgctacagggcgcgtccattcgccattcaggctgcgcaactgttgggaagggcgatcggtgcgggcctcttcgctattacgccagctggcgaaagggggatgtgctgcaaggcgattaagttgggtaacgccagggttttcccagtcacgacgttgtaaaacgacggccagtgaattgtaatacgactcactatagggcgaattgggcccgacgtcgcatgcttggaagggctaattcactcccaaagaagacaagatatccttgatctgtggatctaccacacacaaggctacttccctgattagcagaactacacaccagggccaggggtcagatatccactgacctttggatggtgctacaagctagtaccagttgagccagataaggtagaagaggccaataaaggagagaacaccagcttgttacaccctgtgagcctgcatgggatggatgacccggagagagaagtgttagagtggaggtttgacagccgcctagcatttcatcacgtggcccgagagctgcatccggagtacttcaagaactgctgatatcgagcttgctacaagggactttccgctggggactttccagggaggcgtggcctgggcgggactggggagtggcgagccctcagatcctgcatataagcagctgctttttgcctgtactgggtctctctggttagaccagatctgagcctgggagctctctggctaactagggaacccactgcttaagcctcaataaagcttgccttgagtgcttcaagtagtgtgtgcccgtctgttgtgtgactctggtaactagagatccctcagacccttttagtcagtgtggaaaatctctagcagtggcgcccgaacagggacttgaaagcgaaagggaaaccagaggagctctctcgacgcaggactcggcttgctgaagcgcgcacggcaagaggcgaggggcggcgactggtgagtacgccaaaaattttgactagcggaggctagaaggagagagatgggtgcgagagcgtcagtattaagcgggggagaattagatcgcgatgggaaaaaattcggttaaggccagggggaaagaaaaaatataaattaaaacatatagtatgggcaagcagggagctagaacgattcgcagttaatcctggcctgttagaaacatcagaaggctgtagacaaatactgggacagctacaaccatcccttcagacaggatcagaagaacttagatcattatataatacagtagcaaccctctattgtgtgcatcaaaggatagagataaaagacaccaaggaagctttagacaagatagaggaagagcaaaacaaaagtaagaccaccgcacagcaagcggccgctgatcttcagacctggaggaggagatatgagggacaattggagaagtgaattatataaatataaagtagtaaaaattgaaccattaggagtagcacccaccaaggcaaagagaagagtggtgcagagagaaaaaagagcagtgggaataggagctttgttccttgggttcttgggagcagcaggaagcactatgggcgcagcgtcaatgacgctgacggtacaggccagacaattattgtctggtatagtgcagcagcagaacaatttgctgagggctattgaggcgcaacagcatctgttgcaactcacagtctggggcatcaagcagctccaggcaagaatcctggctgtggaaagatacctaaaggatcaacagctcctggggatttggggttgctctggaaaactcatttgcaccactgctgtgccttggaatgctagttggagtaataaatctctggaacagatttggaatcacacgacctggatggagtgggacagagaaattaacaattacacaagcttaatacactccttaattgaagaatcgcaaaaccagcaagaaaagaatgaacaagaattattggaattagataaatgggcaagtttgtggaattggtttaacataacaaattggctgtggtatataaaattattcataatgatagtaggaggcttggtaggtttaagaatagtttttgctgtactttctatagtgaatagagttaggcagggatattcaccattatcgtttcagacccacctcccaaccccgaggggacccgacaggcccgaaggaatagaagaagaaggtggagagagagacagagacagatccattcgattagtgaacggatctcgacgggatcgattttaaaagaaaaggggggattggggggtacagtgcaggggaaagaatagtagacataatagcaacagacatacaaactaaagaattacaaaaacaaattacaaaaattcaaaattttatcgataagctttgcaaagatggataaagttttaaacagagaggaatctttgcagctaatggaccttctaggtcttgaaaggagtgggaattggctccggtgcccgtcagtgggcagagcgcacatcgcccacagtccccgagaagttggggggaggggtcggcaattgaaccggtgcctagagaaggtggcgcggggtaaactgggaaagtgatgtcgtgtactggctccgcctttttcccgagggtgggggagaaccgtatataagtgcagtagtcgccgtgaacgttctttttcgcaacgggtttgccgccagaacacaggtaagtgccgtgtgtggttcccgcgggcctggcctctttacgggttatggcccttgcgtgccttgaattacttccacctggctgcagtacgtgattcttgatcccgagcttcgggttggaagtgggtgggagagttcgaggccttgcgcttaaggagccccttcgcctcgtgcttgagttgaggcctggcctgggcgctggggccgccgcgtgcgaatctggtggcaccttcgcgcctgtctcgctgctttcgataagtctctagccatttaaaatttttgatgacctgctgcgacgctttttttctggcaagatagtcttgtaaatgcgggccaagatctgcacactggtatttcggtttttggggccgcgggcggcgacggggcccgtgcgtcccagcgcacatgttcggcgaggcggggcctgcgagcgcggccaccgagaatcggacgggggtagtctcaagctggccggcctgctctggtgcctggcctcgcgccgccgtgtatcgccccgccctgggcggcaaggctggcccggtcggcaccagttgcgtgagcggaaagatggccgcttcccggccctgctgcagggagctcaaaatggaggacgcggcgctcgggagagcgggcgggtgagtcacccacacaaaggaaaagggcctttccgtcctcagccgtcgcttcatgtgactccacggagtaccgggcgccgtccaggcacctcgattagttctcgagcttttggagtacgtcgtctttaggttggggggaggggttttatgcgatggagtttccccacactgagtgggtggagactgaagttaggccagcttggcacttgatgtaattctccttggaatttgccctttttgagtttggatcttggttcattctcaagcctcagacagtggttcaaagtttttttcttccatttcaggtgtcgtgaggaattcgctagcgccaccatggagttctcaagcccctctcgggaagaatgcccaaaacctctgtcacgggtgtctatcatggctggatcactgactggcctgctgctgctgcaggccgtgagctgggcctccggagcccggccttgcatcccaaagtctttcggctacagctccgtggtgtgcgtgtgcaacgccacctattgtgactccttcgatccccctacctttcccgccctgggcacattttctcggtacgagtctacacgcagcggcaggagaatggagctgagcatgggccctatccaggccaatcacaccggaacaggcctgctgctgaccctgcagccagagcagaagttccagaaggtgaagggctttggaggagcaatgacagacgcagccgccctgaacatcctggccctgtccccacccgcccagaatctgctgctgaagtcctacttctctgaggagggcatcggctataacatcatcagggtgcccatggccagctgcgacttttccatcagaacctacacatatgccgatacccctgacgatttccagctgcacaatttttccctgccagaggaggatacaaagctgaagatcccactgatccacagggccctgcagctggcccagaggcccgtgagcctgctggccagcccctggacctcccctacatggctgaagaccaacggcgccgtgaatggcaagggctctctgaagggacagccaggcgacatctaccaccagacatgggcccgctatttcgtgaagtttctggatgcctacgccgagcacaagctgcagttctgggccgtgaccgcagagaacgagccttctgccggcctgctgagcggctatcccttccagtgcctgggctttacacctgagcaccagagggactttatcgccagagatctgggcccaaccctggccaactccacacaccacaatgtgcggctgctgatgctggacgatcagcgcctgctgctgcctcactgggccaaggtggtgctgaccgacccagaggccgccaagtacgtgcacggcatcgccgtgcactggtatctggatttcctggcaccagcaaaggccaccctgggagagacacacaggctgttccctaacaccatgctgtttgccagcgaggcctgcgtgggctccaagttttgggagcagtccgtgcggctgggctcttgggacaggggcatgcagtactcccactctatcatcaccaatctgctgtatcacgtggtgggctggacagactggaacctggccctgaatccagagggcggccccaactgggtgagaaatttcgtggatagccccatcatcgtggacatcaccaaggatacattctacaagcagccaatgttttatcacctgggccacttctctaagtttatcccagagggcagccagagggtgggcctggtggccagccagaagaacgacctggatgcagtggccctgatgcaccctgacggctccgccgtggtggtggtgctgaatcgctctagcaaggacgtgcctctgaccatcaaggaccccgccgtgggctttctggagaccatttcacccggctattctattcatacctatctgtggaggaggcagtaacctgcaggggatccaagcttcaattgtggtcactcgacaatcaacctctggattacaaaatttgtgaaagattgactggtattcttaactatgttgctccttttacgctatgtggatacgctgctttaatgcctttgtatcatgctattgcttcccgtatggctttcattttctcctccttgtataaatcctggttgctgtctctttatgaggagttgtggcccgttgtcaggcaacgtggcgtggtgtgcactgtgtttgctgacgcaacccccactggttggggcattgccaccacctgtcagctcctttccgggactttcgctttccccctccctattgccacggcggaactcatcgccgcctgccttgcccgctgctggacaggggctcggctgttgggcactgacaattccgtggtgttgtcggggaagctgacgtcctttccatggctgctcgcctgtgttgccacctggattctgcgcgggacgtccttctgctacgtcccttcggccctcaatccagcggaccttccttcccgcggcctgctgccggctctgcggcctcttccgcgtcttcgccttcgccctcagacgagtcggatctccctttgggccgcctccccgcctgctcgagacctagaaaaacatggagcaatcacaagtagcaatacagcagctaccaatgctgattgtgcctggctagaagcacaagaggaggaggaggtgggttttccagtcacacctcaggtacctttaagaccaatgacttacaaggcagctgtagatcttagccactttttaaaagaaaaggggggactggaagggctaattcactcccaacgaagacaagatctgctttttgcttgtactgggtctctctggttagaccagatctgagcctgggagctctctggctaactagggaacccactgcttaagcctcaataaagcttgccttgagtgcttcaagtagtgtgtgcccgtctgttgtgtgactctggtaactagagatccctcagacccttttagtcagtgtggaaaatctctagcagtagtagttcatgtcatcttattattcagtatttataacttgcaaagaaatgaatatcagagagtgagaggacgcgttggatgcatagcttgagtattctatagtgtcacctaaatagcttggcgtaatcatggtcatagctgtttcctgtgtgaaattgttatccgctcacaattccacacaacatacgagccggaagcataaagtgtaaagcctggggtgcctaatgagtgagctaactcacattaattgcgttgcgctcactgcccgctttccagtcgggaaacctgtcgtgccagctgcattaatgaatcggccaacgcgcggggagaggcggtttgcgtattgggcgctcttccgcttcctcgctcactgactcgctgcgctcggtcgttcggctgcggcgagcggtatcagctcactcaaaggcggtaatacggttatccacagaatcaggggataacgcaggaaagaacatgtgagcaaaaggccagcaaaaggccaggaaccgtaaaaaggccgcgttgctggcgtttttccataggctccgcccccctgacgagcatcacaaaaatcgacgctcaagtcagaggtggcgaaacccgacaggactataaagataccaggcgtttccccctggaagctccctcgtgcgctctcctgttccgaccctgccgcttaccggatacctgtccgcctttctcccttcgggaagcgtggcgctttctcatagctcacgctgtaggtatctcagttcggtgtaggtcgttcgctccaagctgggctgtgtgcacgaaccccccgttcagcccgaccgctgcgccttatccggtaactatcgtcttgagtccaacccggtaagacacgacttatcgccactggcagcagccactggtaacaggattagcagagcgaggtatgtaggcggtgctacagagttcttgaagtggtggcctaactacggctacactagaagaacagtatttggtatctgcgctctgctgaagccagttaccttcggaaaaagagttggtagctcttgatccggcaaacaaaccaccgctggtagcggtggtttttttgtttgcaagcagcagattacgcgcagaaaaaaaggatctcaagaagatcctttgatcttttctacggggtctgacgctcagtggaacgaaaactcacgttaagggattttggtcatgagattatcaaaaaggatcttcacctagatccttttaaattaaaaatgaagttttaaatcaatctaaagtatatatgagtaaacttggtctgacagttaccaatgcttaatcagtgaggcacctatctcagcgatctgtctatttcgttcatccatagttgcctgactccccgtcgtgtagataactacgatacgggagggcttaccatctggccccagtgctgcaatgataccgcgagacccacgctcaccggctccagatttatcagcaataaaccagccagccggaagggccgagcgcagaagtggtcctgcaactttatccgcctccatccagtctattaattgttgccgggaagctagagtaagtagttcgccagttaatagtttgcgcaacgttgttgccattgctacaggcatcgtggtgtcacgctcgtcgtttggtatggcttcattcagctccggttcccaacgatcaaggcgagttacatgatcccccatgttgtgcaaaaaagcggttagctccttcggtcctccgatcgttgtcagaagtaagttggccgcagtgttatcactcatggttatggcagcactgcataattctcttactgtcatgccatccgtaagatgcttttctgtgactggtgagtactcaaccaagtcattctgagaatagtgtatgcggcgaccgagttgctcttgcccggcgtcaatacgggataataccgcgccacatagcagaactttaaaagtgctcatcattggaaaacgttcttcggggcgaaaactctcaaggatcttaccgctgttgagatccagttcgatgtaacccactcgtgcacccaactgatcttcagcatcttttactttcaccagcgtttctgggtgagcaaaaacaggaaggcaaaatgccgcaaaaaagggaataagggcgacacggaaatgttgaatactcatactcttcctttttcaatattattgaagcatttatcagggttattgtctcatgagcggatacatatttgaatgtatttagaaaaataaacaaataggggttccgcgcacatttccccgaaaagtgccacctgatgcggtgtgaaataccgcacagatgcgtaaggagaaaataccgcatcagg

SEQ ID NO: 5 - DNA, 8681 bp, Artificial Sequence
  Lentiviral vector comprising ASAH1 transgene
gggcgaattgggcccgacgtcgcatgcttggaagggctaattcactcccaaagaagacaagatatccttgatctgtggatctaccacacacaaggctacttccctgattagcagaactacacaccagggccaggggtcagatatccactgacctttggatggtgctacaagctagtaccagttgagccagataaggtagaagaggccaataaaggagagaacaccagcttgttacaccctgtgagcctgcatgggatggatgacccggagagagaagtgttagagtggaggtttgacagccgcctagcatttcatcacgtggcccgagagctgcatccggagtacttcaagaactgctgatatcgagcttgctacaagggactttccgctggggactttccagggaggcgtggcctgggcgggactggggagtggcgagccctcagatcctgcatataagcagctgctttttgcctgtactgggtctctctggttagaccagatctgagcctgggagctctctggctaactagggaacccactgcttaagcctcaataaagcttgccttgagtgcttcaagtagtgtgtgcccgtctgttgtgtgactctggtaactagagatccctcagacccttttagtcagtgtggaaaatctctagcagtggcgcccgaacagggacttgaaagcgaaagggaaaccagaggagctctctcgacgcaggactcggcttgctgaagcgcgcacggcaagaggcgaggggcggcgactggtgagtacgccaaaaattttgactagcggaggctagaaggagagagatgggtgcgagagcgtcagtattaagcgggggagaattagatcgcgatgggaaaaaattcggttaaggccagggggaaagaaaaaatataaattaaaacatatagtatgggcaagcagggagctagaacgattcgcagttaatcctggcctgttagaaacatcagaaggctgtagacaaatactgggacagctacaaccatcccttcagacaggatcagaagaacttagatcattatataatacagtagcaaccctctattgtgtgcatcaaaggatagagataaaagacaccaaggaagctttagacaagatagaggaagagcaaaacaaaagtaagaccaccgcacagcaagcggccgctgatcttcagacctggaggaggagatatgagggacaattggagaagtgaattatataaatataaagtagtaaaaattgaaccattaggagtagcacccaccaaggcaaagagaagagtggtgcagagagaaaaaagagcagtgggaataggagctttgttccttgggttcttgggagcagcaggaagcactatgggcgcagcgtcaatgacgctgacggtacaggccagacaattattgtctggtatagtgcagcagcagaacaatttgctgagggctattgaggcgcaacagcatctgttgcaactcacagtctggggcatcaagcagctccaggcaagaatcctggctgtggaaagatacctaaaggatcaacagctcctggggatttggggttgctctggaaaactcatttgcaccactgctgtgccttggaatgctagttggagtaataaatctctggaacagatttggaatcacacgacctggatggagtgggacagagaaattaacaattacacaagcttaatacactccttaattgaagaatcgcaaaaccagcaagaaaagaatgaacaagaattattggaattagataaatgggcaagtttgtggaattggtttaacataacaaattggctgtggtatataaaattattcataatgatagtaggaggcttggtaggtttaagaatagtttttgctgtactttctatagtgaatagagttaggcagggatattcaccattatcgtttcagacccacctcccaaccccgaggggacccgacaggcccgaaggaatagaagaagaaggtggagagagagacagagacagatccattcgattagtgaacggatctcgacgggatcgattttaaaagaaaaggggggattggggggtacagtgcaggggaaagaatagtagacataatagcaacagacatacaaactaaagaattacaaaaacaaattacaaaaattcaaaattttatcgataagctttgcaaagatggataaagttttaaacagagaggaatctttgcagctaatggaccttctaggtcttgaaaggagtgggaattggctccggtgcccgtcagtgggcagagcgcacatcgcccacagtccccgagaagttggggggaggggtcggcaattgaaccggtgcctagagaaggtggcgcggggtaaactgggaaagtgatgtcgtgtactggctccgcctttttcccgagggtgggggagaaccgtatataagtgcagtagtcgccgtgaacgttctttttcgcaacgggtttgccgccagaacacaggtaagtgccgtgtgtggttcccgcgggcctggcctctttacgggttatggcccttgcgtgccttgaattacttccacctggctgcagtacgtgattcttgatcccgagcttcgggttggaagtgggtgggagagttcgaggccttgcgcttaaggagccccttcgcctcgtgcttgagttgaggcctggcctgggcgctggggccgccgcgtgcgaatctggtggcaccttcgcgcctgtctcgctgctttcgataagtctctagccatttaaaatttttgatgacctgctgcgacgctttttttctggcaagatagtcttgtaaatgcgggccaagatctgcacactggtatttcggtttttggggccgcgggcggcgacggggcccgtgcgtcccagcgcacatgttcggcgaggcggggcctgcgagcgcggccaccgagaatcggacgggggtagtctcaagctggccggcctgctctggtgcctggcctcgcgccgccgtgtatcgccccgccctgggcggcaaggctggcccggtcggcaccagttgcgtgagcggaaagatggccgcttcccggccctgctgcagggagctcaaaatggaggacgcggcgctcgggagagcgggcgggtgagtcacccacacaaaggaaaagggcctttccgtcctcagccgtcgcttcatgtgactccacggagtaccgggcgccgtccaggcacctcgattagttctcgagcttttggagtacgtcgtctttaggttggggggaggggttttatgcgatggagtttccccacactgagtgggtggagactgaagttaggccagcttggcacttgatgtaattctccttggaatttgccctttttgagtttggatcttggttcattctcaagcctcagacagtggttcaaagtttttttcttccatttcaggtgtcgtgaggaattctgcagtcgacgccaccatgccgggccggagttgcgtcgccttagtcctcctggctgccgccgtcagctgtgccgtcgcgcagcacgcgccgccgtggacagaggactgcagaaaatcaacctatcctccttcaggaccaacgtacagaggtgcagttccatggtacaccataaatcttgacttaccaccctacaaaagatggcatgaattgatgcttgacaaggcaccagtgctaaaggttatagtgaattctctgaagaatatgataaatacattcgtgccaagtggaaaaattatgcaggtggtggatgaaaaattgcctggcctacttggcaactttcctggcccttttgaagaggaaatgaagggtattgccgctgttactgatatacctttaggagagattatttcattcaatattttttatgaattatttaccatttgtacttcaatagtagcagaagacaaaaaaggtcatctaatacatgggagaaacatggattttggagtatttcttgggtggaacataaataatgatacctgggtcataactgagcaactaaaacctttaacagtgaatttggatttccaaagaaacaacaaaactgtcttcaaggcttcaagctttgctggctatgtgggcatgttaacaggattcaaaccaggactgttcagtcttacactgaatgaacgtttcagtataaatggtggttatctgggtattctagaatggattctgggaaagaaagatgtcatgtggatagggttcctcactagaacagttctggaaaatagcacaagttatgaagaagccaagaatttattgaccaagaccaagatattggccccagcctactttatcctgggaggcaaccagtctggggaaggttgtgtgattacacgagacagaaaggaatcattggatgtatatgaactcgatgctaagcagggtagatggtatgtggtacaaacaaattatgaccgttggaaacatcccttcttccttgatgatcgcagaacgcctgcaaagatgtgtctgaaccgcaccagccaagagaatatctcatttgaaaccatgtatgatgtcctgtcaacaaaacctgtcctcaacaagctgaccgtatacacaaccttgatagatgttaccaaaggtcaattcgaaacttacctgcgggactgccctgacccttgtataggttggtgagcggccgcctcgaggatccaagcttcaattgtggtcactcgacaatcaacctctggattacaaaatttgtgaaagattgactggtattcttaactatgttgctccttttacgctatgtggatacgctgctttaatgcctttgtatcatgctattgcttcccgtatggctttcattttctcctccttgtataaatcctggttgctgtctctttatgaggagttgtggcccgttgtcaggcaacgtggcgtggtgtgcactgtgtttgctgacgcaacccccactggttggggcattgccaccacctgtcagctcctttccgggactttcgctttccccctccctattgccacggcggaactcatcgccgcctgccttgcccgctgctggacaggggctcggctgttgggcactgacaattccgtggtgttgtcggggaagctgacgtcctttccatggctgctcgcctgtgttgccacctggattctgcgcgggacgtccttctgctacgtcccttcggccctcaatccagcggaccttccttcccgcggcctgctgccggctctgcggcctcttccgcgtcttcgccttcgccctcagacgagtcggatctccctttgggccgcctccccgcctgctcgagacctagaaaaacatggagcaatcacaagtagcaatacagcagctaccaatgctgattgtgcctggctagaagcacaagaggaggaggaggtgggttttccagtcacacctcaggtacctttaagaccaatgacttacaaggcagctgtagatcttagccactttttaaaagaaaaggggggactggaagggctaattcactcccaacgaagacaagatctgctttttgcttgtactgggtctctctggttagaccagatctgagcctgggagctctctggctaactagggaacccactgcttaagcctcaataaagcttgccttgagtgcttcaagtagtgtgtgcccgtctgttgtgtgactctggtaactagagatccctcagacccttttagtcagtgtggaaaatctctagcagtagtagttcatgtcatcttattattcagtatttataacttgcaaagaaatgaatatcagagagtgagaggacgcgttggatgcatagcttgagtattctatagtgtcacctaaatagcttggcgtaatcatggtcatagctgtttcctgtgtgaaattgttatccgctcacaattccacacaacatacgagccggaagcataaagtgtaaagcctggggtgcctaatgagtgagctaactcacattaattgcgttgcgctcactgcccgctttccagtcgggaaacctgtcgtgccagctgcattaatgaatcggccaacgcgcggggagaggcggtttgcgtattgggcgctcttccgcttcctcgctcactgactcgctgcgctcggtcgttcggctgcggcgagcggtatcagctcactcaaaggcggtaatacggttatccacagaatcaggggataacgcaggaaagaacatgtgagcaaaaggccagcaaaaggccaggaaccgtaaaaaggccgcgttgctggcgtttttccataggctccgcccccctgacgagcatcacaaaaatcgacgctcaagtcagaggtggcgaaacccgacaggactataaagataccaggcgtttccccctggaagctccctcgtgcgctctcctgttccgaccctgccgcttaccggatacctgtccgcctttctcccttcgggaagcgtggcgctttctcatagctcacgctgtaggtatctcagttcggtgtaggtcgttcgctccaagctgggctgtgtgcacgaaccccccgttcagcccgaccgctgcgccttatccggtaactatcgtcttgagtccaacccggtaagacacgacttatcgccactggcagcagccactggtaacaggattagcagagcgaggtatgtaggcggtgctacagagttcttgaagtggtggcctaactacggctacactagaagaacagtatttggtatctgcgctctgctgaagccagttaccttcggaaaaagagttggtagctcttgatccggcaaacaaaccaccgctggtagcggtggtttttttgtttgcaagcagcagattacgcgcagaaaaaaaggatctcaagaagatcctttgatcttttctacggggtctgacgctcagtggaacgaaaactcacgttaagggattttggtcatgagattatcaaaaaggatcttcacctagatccttttaaattaaaaatgaagttttaaatcaatctaaagtatatatgagtaaacttggtctgacagttaccaatgcttaatcagtgaggcacctatctcagcgatctgtctatttcgttcatccatagttgcctgactccccgtcgtgtagataactacgatacgggagggcttaccatctggccccagtgctgcaatgataccgcgagacccacgctcaccggctccagatttatcagcaataaaccagccagccggaagggccgagcgcagaagtggtcctgcaactttatccgcctccatccagtctattaattgttgccgggaagctagagtaagtagttcgccagttaatagtttgcgcaacgttgttgccattgctacaggcatcgtggtgtcacgctcgtcgtttggtatggcttcattcagctccggttcccaacgatcaaggcgagttacatgatcccccatgttgtgcaaaaaagcggttagctccttcggtcctccgatcgttgtcagaagtaagttggccgcagtgttatcactcatggttatggcagcactgcataattctcttactgtcatgccatccgtaagatgcttttctgtgactggtgagtactcaaccaagtcattctgagaatagtgtatgcggcgaccgagttgctcttgcccggcgtcaatacgggataataccgcgccacatagcagaactttaaaagtgctcatcattggaaaacgttcttcggggcgaaaactctcaaggatcttaccgctgttgagatccagttcgatgtaacccactcgtgcacccaactgatcttcagcatcttttactttcaccagcgtttctgggtgagcaaaaacaggaaggcaaaatgccgcaaaaaagggaataagggcgacacggaaatgttgaatactcatactcttcctttttcaatattattgaagcatttatcagggttattgtctcatgagcggatacatatttgaatgtatttagaaaaataaacaaataggggttccgcgcacatttccccgaaaagtgccacctgatgcggtgtgaaataccgcacagatgcgtaaggagaaaataccgcatcaggaaattgtaagcgttaatattttgttaaaattcgcgttaaatttttgttaaatcagctcattttttaaccaataggccgaaatcggcaaaatcccttataaatcaaaagaatagaccgagatagggttgagtgttgttccagtttggaacaagagtccactattaaagaacgtggactccaacgtcaaagggcgaaaaaccgtctatcagggcgatggcccactacgtgaaccatcaccctaatcaagttttttggggtcgaggtgccgtaaagcactaaatcggaaccctaaagggagcccccgatttagagcttgacggggaaagccggcgaacgtggcgagaaaggaagggaagaaagcgaaaggagcgggcgctagggcgctggcaagtgtagcggtcacgctgcgcgtaaccaccacacccgccgcgcttaatgcgccgctacagggcgcgtccattcgccattcaggctgcgcaactgttgggaagggcgatcggtgcgggcctcttcgctattacgccagctggcgaaagggggatgtgctgcaaggcgattaagttgggtaacgccagggttttcccagtcacgacgttgtaaaacgacggccagtgaattgtaatacgactcactata

SEQ ID NO: 6 - DNA, 10336 bp, Artificial Sequence
  Lentiviral vector comprising GAA transgene
aaattgtaagcgttaatattttgttaaaattcgcgttaaatttttgttaaatcagctcattttttaaccaataggccgaaatcggcaaaatcccttataaatcaaaagaatagaccgagatagggttgagtgttgttccagtttggaacaagagtccactattaaagaacgtggactccaacgtcaaagggcgaaaaaccgtctatcagggcgatggcccactacgtgaaccatcaccctaatcaagttttttggggtcgaggtgccgtaaagcactaaatcggaaccctaaagggagcccccgatttagagcttgacggggaaagccggcgaacgtggcgagaaaggaagggaagaaagcgaaaggagcgggcgctagggcgctggcaagtgtagcggtcacgctgcgcgtaaccaccacacccgccgcgcttaatgcgccgctacagggcgcgtccattcgccattcaggctgcgcaactgttgggaagggcgatcggtgcgggcctcttcgctattacgccagctggcgaaagggggatgtgctgcaaggcgattaagttgggtaacgccagggttttcccagtcacgacgttgtaaaacgacggccagtgaattgtaatacgactcactatagggcgaattgggcccgacgtcgcatgcttggaagggctaattcactcccaaagaagacaagatatccttgatctgtggatctaccacacacaaggctacttccctgattagcagaactacacaccagggccaggggtcagatatccactgacctttggatggtgctacaagctagtaccagttgagccagataaggtagaagaggccaataaaggagagaacaccagcttgttacaccctgtgagcctgcatgggatggatgacccggagagagaagtgttagagtggaggtttgacagccgcctagcatttcatcacgtggcccgagagctgcatccggagtacttcaagaactgctgatatcgagcttgctacaagggactttccgctggggactttccagggaggcgtggcctgggcgggactggggagtggcgagccctcagatcctgcatataagcagctgctttttgcctgtactgggtctctctggttagaccagatctgagcctgggagctctctggctaactagggaacccactgcttaagcctcaataaagcttgccttgagtgcttcaagtagtgtgtgcccgtctgttgtgtgactctggtaactagagatccctcagacccttttagtcagtgtggaaaatctctagcagtggcgcccgaacagggacttgaaagcgaaagggaaaccagaggagctctctcgacgcaggactcggcttgctgaagcgcgcacggcaagaggcgaggggcggcgactggtgagtacgccaaaaattttgactagcggaggctagaaggagagagatgggtgcgagagcgtcagtattaagcgggggagaattagatcgcgatgggaaaaaattcggttaaggccagggggaaagaaaaaatataaattaaaacatatagtatgggcaagcagggagctagaacgattcgcagttaatcctggcctgttagaaacatcagaaggctgtagacaaatactgggacagctacaaccatcccttcagacaggatcagaagaacttagatcattatataatacagtagcaaccctctattgtgtgcatcaaaggatagagataaaagacaccaaggaagctttagacaagatagaggaagagcaaaacaaaagtaagaccaccgcacagcaagcggccgctgatcttcagacctggaggaggagatatgagggacaattggagaagtgaattatataaatataaagtagtaaaaattgaaccattaggagtagcacccaccaaggcaaagagaagagtggtgcagagagaaaaaagagcagtgggaataggagctttgttccttgggttcttgggagcagcaggaagcactatgggcgcagcgtcaatgacgctgacggtacaggccagacaattattgtctggtatagtgcagcagcagaacaatttgctgagggctattgaggcgcaacagcatctgttgcaactcacagtctggggcatcaagcagctccaggcaagaatcctggctgtggaaagatacctaaaggatcaacagctcctggggatttggggttgctctggaaaactcatttgcaccactgctgtgccttggaatgctagttggagtaataaatctctggaacagatttggaatcacacgacctggatggagtgggacagagaaattaacaattacacaagcttaatacactccttaattgaagaatcgcaaaaccagcaagaaaagaatgaacaagaattattggaattagataaatgggcaagtttgtggaattggtttaacataacaaattggctgtggtatataaaattattcataatgatagtaggaggcttggtaggtttaagaatagtttttgctgtactttctatagtgaatagagttaggcagggatattcaccattatcgtttcagacccacctcccaaccccgaggggacccgacaggcccgaaggaatagaagaagaaggtggagagagagacagagacagatccattcgattagtgaacggatctcgacgggatcgattttaaaagaaaaggggggattggggggtacagtgcaggggaaagaatagtagacataatagcaacagacatacaaactaaagaattacaaaaacaaattacaaaaattcaaaattttatcgataagctttgcaaagatggataaagttttaaacagagaggaatctttgcagctaatggaccttctaggtcttgaaaggagtgggaattggctccggtgcccgtcagtgggcagagcgcacatcgcccacagtccccgagaagttggggggaggggtcggcaattgaaccggtgcctagagaaggtggcgcggggtaaactgggaaagtgatgtcgtgtactggctccgcctttttcccgagggtgggggagaaccgtatataagtgcagtagtcgccgtgaacgttctttttcgcaacgggtttgccgccagaacacaggtaagtgccgtgtgtggttcccgcgggcctggcctctttacgggttatggcccttgcgtgccttgaattacttccacctggctgcagtacgtgattcttgatcccgagcttcgggttggaagtgggtgggagagttcgaggccttgcgcttaaggagccccttcgcctcgtgcttgagttgaggcctggcctgggcgctggggccgccgcgtgcgaatctggtggcaccttcgcgcctgtctcgctgctttcgataagtctctagccatttaaaatttttgatgacctgctgcgacgctttttttctggcaagatagtcttgtaaatgcgggccaagatctgcacactggtatttcggtttttggggccgcgggcggcgacggggcccgtgcgtcccagcgcacatgttcggcgaggcggggcctgcgagcgcggccaccgagaatcggacgggggtagtctcaagctggccggcctgctctggtgcctggcctcgcgccgccgtgtatcgccccgccctgggcggcaaggctggcccggtcggcaccagttgcgtgagcggaaagatggccgcttcccggccctgctgcagggagctcaaaatggaggacgcggcgctcgggagagcgggcgggtgagtcacccacacaaaggaaaagggcctttccgtcctcagccgtcgcttcatgtgactccacggagtaccgggcgccgtccaggcacctcgattagttctcgagcttttggagtacgtcgtctttaggttggggggaggggttttatgcgatggagtttccccacactgagtgggtggagactgaagttaggccagcttggcacttgatgtaattctccttggaatttgccctttttgagtttggatcttggttcattctcaagcctcagacagtggttcaaagtttttttcttccatttcaggtgtcgtgaggaattcgccaccatgggcgtgaggcaccccccttgctctcacaggctgctggccgtgtgcgcactggtgagcctggccaccgccgccctgctgggccacatcctgctgcacgacttcctgctggtgcccagggagctgtccggcagctccccagtgctggaggagacccacccagcacaccagcagggcgcctctcggccaggcccccgcgatgcacaggcacacccaggccggccccgcgccgtgccaacccagtgcgacgtgccacccaacagccggtttgactgtgcccccgataaggccatcacacaggagcagtgcgaggccaggggctgctgttatatccctgcaaagcagggcctccagggcgcccagatgggacagccatggtgtttctttcctccatcttaccccagctataagctggagaatctgtctagctccgagatgggctacacagccaccctgacaagaaccacaccaacattctttcccaaggacatcctgaccctgcggctggacgtgatgatggagacagagaaccgcctgcacttcaccatcaaggaccccgccaataggagatatgaggtgcctctggagaccccacacgtgcactctcgggcccctagcccactgtactccgtggagttctctgaggagccatttggcgtgatcgtgcggcgccagctggatggacgcgtgctgctgaacaccacagtggcccccctgttctttgccgaccagttcctccagctgagcacatccctgccctcccagtatatcaccggcctggccgagcacctgtctcctctgatgctgtctaccagctggacaaggatcaccctgtggaacagagacctggcaccaacccctggcgcaaatctgtacggcagccaccctttctatctggccctggaggatggaggctccgcccacggcgtgtttctgctgaactctaatgccatggacgtggtgctccagccaagccccgccctgtcctggcggtctaccggcggcatcctggacgtgtacatcttcctgggccctgagccaaagtccgtggtgcagcagtacctggacgtggtgggctatcctttcatgcccccttactggggactgggatttcacctgtgccgctggggctattctagcacagccatcacccggcaggtggtggagaacatgacccgcgcccactttccactggatgtgcagtggaatgacctggattacatggactccaggagagacttcaccttcaacaaggacggcttcagggattttcccgccatggtgcaggagctgcaccagggcggccggcgctacatgatgatcgtggaccccgccatctcctctagcggacctgccggcagctacagaccatatgacgagggcctgaggagaggcgtgttcatcacaaacgagaccggccagcctctgatcggcaaggtctggccaggctccaccgccttcccagacttcaccaatccaaccgccctggcctggtgggaggacatggtggccgagttccacgaccaggtgccttttgatggcatgtggatcgacatgaacgagccatctaatttcatcaggggcagcgaggacggctgccccaacaatgagctggagaacccaccatatgtgcctggcgtggtgggaggcaccctccaggcagcaaccatctgtgcctcctctcaccagtttctgtctacacactataacctgcacaatctgtacggactgaccgaggcaatcgccagccacagagccctggtgaaggccaggggcacaagacctttcgtgatctccaggtctacctttgccggacacggcagatacgcaggacactggaccggcgacgtgtggagcagctgggagcagctggcctctagcgtgccagagatcctccagttcaacctgctgggcgtgcccctggtgggagcagacgtgtgcggctttctgggcaatacatccgaggagctgtgcgtgaggtggacccagctgggagccttctatcccttcatgcgcaaccacaatagcctgctgtccctgcctcaggagccatacagcttctccgagcctgcacagcaggcaatgaggaaggccctgacactgcgctatgccctgctgccacacctgtacaccctgtttcaccaggcacacgtggcaggagagacagtggcccggcccctgttcctggagtttcctaaggattcctctacctggacagtggaccaccagctgctgtggggagaggccctgctgatcacccccgtgctccaggcaggcaaggcagaggtgacaggctatttccctctgggcacatggtacgacctccagaccgtgccagtggaggccctgggcagcctgcctccaccacctgccgccccccgcgagcctgccatccactccgagggacagtgggtgacactgccagcacctctggacaccatcaacgtgcacctgagggccggctatatcatccccctccagggccctggcctgaccacaaccgagtccagacagcagccaatggccctggccgtggccctgaccaagggaggcgaggccaggggcgagctgttctgggacgatggcgagtctctggaggtgctggagagaggcgcctacacacaggtcatcttcctggccaggaacaatacaatcgtgaatgagctggtgagagtgacctctgagggagcaggactccagctccagaaggtgacagtgctgggagtggcaaccgcaccacagcaggtgctgagcaacggcgtgcccgtgagcaatttcacatactcccctgataccaaggtgctggacatctgcgtgagcctgctgatgggcgagcagtttctggtgtcctggtgttgagaacccgggatccaagcttcaattgtggtcactcgacaatcaacctctggattacaaaatttgtgaaagattgactggtattcttaactatgttgctccttttacgctatgtggatacgctgctttaatgcctttgtatcatgctattgcttcccgtatggctttcattttctcctccttgtataaatcctggttgctgtctctttatgaggagttgtggcccgttgtcaggcaacgtggcgtggtgtgcactgtgtttgctgacgcaacccccactggttggggcattgccaccacctgtcagctcctttccgggactttcgctttccccctccctattgccacggcggaactcatcgccgcctgccttgcccgctgctggacaggggctcggctgttgggcactgacaattccgtggtgttgtcggggaagctgacgtcctttccatggctgctcgcctgtgttgccacctggattctgcgcgggacgtccttctgctacgtcccttcggccctcaatccagcggaccttccttcccgcggcctgctgccggctctgcggcctcttccgcgtcttcgccttcgccctcagacgagtcggatctccctttgggccgcctccccgcctgctcgagacctagaaaaacatggagcaatcacaagtagcaatacagcagctaccaatgctgattgtgcctggctagaagcacaagaggaggaggaggtgggttttccagtcacacctcaggtacctttaagaccaatgacttacaaggcagctgtagatcttagccactttttaaaagaaaaggggggactggaagggctaattcactcccaacgaagacaagatctgctttttgcttgtactgggtctctctggttagaccagatctgagcctgggagctctctggctaactagggaacccactgcttaagcctcaataaagcttgccttgagtgcttcaagtagtgtgtgcccgtctgttgtgtgactctggtaactagagatccctcagacccttttagtcagtgtggaaaatctctagcagtagtagttcatgtcatcttattattcagtatttataacttgcaaagaaatgaatatcagagagtgagaggacgcgttggatgcatagcttgagtattctatagtgtcacctaaatagcttggcgtaatcatggtcatagctgtttcctgtgtgaaattgttatccgctcacaattccacacaacatacgagccggaagcataaagtgtaaagcctggggtgcctaatgagtgagctaactcacattaattgcgttgcgctcactgcccgctttccagtcgggaaacctgtcgtgccagctgcattaatgaatcggccaacgcgcggggagaggcggtttgcgtattgggcgctcttccgcttcctcgctcactgactcgctgcgctcggtcgttcggctgcggcgagcggtatcagctcactcaaaggcggtaatacggttatccacagaatcaggggataacgcaggaaagaacatgtgagcaaaaggccagcaaaaggccaggaaccgtaaaaaggccgcgttgctggcgtttttccataggctccgcccccctgacgagcatcacaaaaatcgacgctcaagtcagaggtggcgaaacccgacaggactataaagataccaggcgtttccccctggaagctccctcgtgcgctctcctgttccgaccctgccgcttaccggatacctgtccgcctttctcccttcgggaagcgtggcgctttctcatagctcacgctgtaggtatctcagttcggtgtaggtcgttcgctccaagctgggctgtgtgcacgaaccccccgttcagcccgaccgctgcgccttatccggtaactatcgtcttgagtccaacccggtaagacacgacttatcgccactggcagcagccactggtaacaggattagcagagcgaggtatgtaggcggtgctacagagttcttgaagtggtggcctaactacggctacactagaagaacagtatttggtatctgcgctctgctgaagccagttaccttcggaaaaagagttggtagctcttgatccggcaaacaaaccaccgctggtagcggtggtttttttgtttgcaagcagcagattacgcgcagaaaaaaaggatctcaagaagatcctttgatcttttctacggggtctgacgctcagtggaacgaaaactcacgttaagggattttggtcatgagattatcaaaaaggatcttcacctagatccttttaaattaaaaatgaagttttaaatcaatctaaagtatatatgagtaaacttggtctgacagttaccaatgcttaatcagtgaggcacctatctcagcgatctgtctatttcgttcatccatagttgcctgactccccgtcgtgtagataactacgatacgggagggcttaccatctggccccagtgctgcaatgataccgcgagacccacgctcaccggctccagatttatcagcaataaaccagccagccggaagggccgagcgcagaagtggtcctgcaactttatccgcctccatccagtctattaattgttgccgggaagctagagtaagtagttcgccagttaatagtttgcgcaacgttgttgccattgctacaggcatcgtggtgtcacgctcgtcgtttggtatggcttcattcagctccggttcccaacgatcaaggcgagttacatgatcccccatgttgtgcaaaaaagcggttagctccttcggtcctccgatcgttgtcagaagtaagttggccgcagtgttatcactcatggttatggcagcactgcataattctcttactgtcatgccatccgtaagatgcttttctgtgactggtgagtactcaaccaagtcattctgagaatagtgtatgcggcgaccgagttgctcttgcccggcgtcaatacgggataataccgcgccacatagcagaactttaaaagtgctcatcattggaaaacgttcttcggggcgaaaactctcaaggatcttaccgctgttgagatccagttcgatgtaacccactcgtgcacccaactgatcttcagcatcttttactttcaccagcgtttctgggtgagcaaaaacaggaaggcaaaatgccgcaaaaaagggaataagggcgacacggaaatgttgaatactcatactcttcctttttcaatattattgaagcatttatcagggttattgtctcatgagcggatacatatttgaatgtatttagaaaaataaacaaataggggttccgcgcacatttccccgaaaagtgccacctgatgcggtgtgaaataccgcacagatgcgtaaggagaaaataccgcatcagg

SEQ ID NO: 7 - DNA, 1611 bp, Artificial Sequence
  GBA transgene
atggagttctcaagcccctctcgggaagaatgcccaaaacctctgtcacgggtgtctatcatggctggatcactgactggcctgctgctgctgcaggccgtgagctgggcctccggagcccggccttgcatcccaaagtctttcggctacagctccgtggtgtgcgtgtgcaacgccacctattgtgactccttcgatccccctacctttcccgccctgggcacattttctcggtacgagtctacacgcagcggcaggagaatggagctgagcatgggccctatccaggccaatcacaccggaacaggcctgctgctgaccctgcagccagagcagaagttccagaaggtgaagggctttggaggagcaatgacagacgcagccgccctgaacatcctggccctgtccccacccgcccagaatctgctgctgaagtcctacttctctgaggagggcatcggctataacatcatcagggtgcccatggccagctgcgacttttccatcagaacctacacatatgccgatacccctgacgatttccagctgcacaatttttccctgccagaggaggatacaaagctgaagatcccactgatccacagggccctgcagctggcccagaggcccgtgagcctgctggccagcccctggacctcccctacatggctgaagaccaacggcgccgtgaatggcaagggctctctgaagggacagccaggcgacatctaccaccagacatgggcccgctatttcgtgaagtttctggatgcctacgccgagcacaagctgcagttctgggccgtgaccgcagagaacgagccttctgccggcctgctgagcggctatcccttccagtgcctgggctttacacctgagcaccagagggactttatcgccagagatctgggcccaaccctggccaactccacacaccacaatgtgcggctgctgatgctggacgatcagcgcctgctgctgcctcactgggccaaggtggtgctgaccgacccagaggccgccaagtacgtgcacggcatcgccgtgcactggtatctggatttcctggcaccagcaaaggccaccctgggagagacacacaggctgttccctaacaccatgctgtttgccagcgaggcctgcgtgggctccaagttttgggagcagtccgtgcggctgggctcttgggacaggggcatgcagtactcccactctatcatcaccaatctgctgtatcacgtggtgggctggacagactggaacctggccctgaatccagagggcggccccaactgggtgagaaatttcgtggatagccccatcatcgtggacatcaccaaggatacattctacaagcagccaatgttttatcacctgggccacttctctaagtttatcccagagggcagccagagggtgggcctggtggccagccagaagaacgacctggatgcagtggccctgatgcaccctgacggctccgccgtggtggtggtgctgaatcgctctagcaaggacgtgcctctgaccatcaaggaccccgccgtgggctttctggagaccatttcacccggctattctattcatacctatctgtggaggaggcagtaa

SEQ ID NO: 8 - DNA, 1188 bp, Artificial Sequence
  ASAH1 transgene
atgccgggccggagttgcgtcgccttagtcctcctggctgccgccgtcagctgtgccgtcgcgcagcacgcgccgccgtggacagaggactgcagaaaatcaacctatcctccttcaggaccaacgtacagaggtgcagttccatggtacaccataaatcttgacttaccaccctacaaaagatggcatgaattgatgcttgacaaggcaccagtgctaaaggttatagtgaattctctgaagaatatgataaatacattcgtgccaagtggaaaaattatgcaggtggtggatgaaaaattgcctggcctacttggcaactttcctggcccttttgaagaggaaatgaagggtattgccgctgttactgatatacctttaggagagattatttcattcaatattttttatgaattatttaccatttgtacttcaatagtagcagaagacaaaaaaggtcatctaatacatgggagaaacatggattttggagtatttcttgggtggaacataaataatgatacctgggtcataactgagcaactaaaacctttaacagtgaatttggatttccaaagaaacaacaaaactgtcttcaaggcttcaagctttgctggctatgtgggcatgttaacaggattcaaaccaggactgttcagtcttacactgaatgaacgtttcagtataaatggtggttatctgggtattctagaatggattctgggaaagaaagatgtcatgtggatagggttcctcactagaacagttctggaaaatagcacaagttatgaagaagccaagaatttattgaccaagaccaagatattggccccagcctactttatcctgggaggcaaccagtctggggaaggttgtgtgattacacgagacagaaaggaatcattggatgtatatgaactcgatgctaagcagggtagatggtatgtggtacaaacaaattatgaccgttggaaacatcccttcttccttgatgatcgcagaacgcctgcaaagatgtgtctgaaccgcaccagccaagagaatatctcatttgaaaccatgtatgatgtcctgtcaacaaaacctgtcctcaacaagctgaccgtatacacaaccttgatagatgttaccaaaggtcaattcgaaacttacctgcgggactgccctgacccttgtataggttggtga

SEQ ID NO: 9 - DNA, 2859 bp, Artificial Sequence
  GAA transgene
atgggcgtgaggcaccccccttgctctcacaggctgctggccgtgtgcgcactggtgagcctggccaccgccgccctgctgggccacatcctgctgcacgacttcctgctggtgcccagggagctgtccggcagctccccagtgctggaggagacccacccagcacaccagcagggcgcctctcggccaggcccccgcgatgcacaggcacacccaggccggccccgcgccgtgccaacccagtgcgacgtgccacccaacagccggtttgactgtgcccccgataaggccatcacacaggagcagtgcgaggccaggggctgctgttatatccctgcaaagcagggcctccagggcgcccagatgggacagccatggtgtttctttcctccatcttaccccagctataagctggagaatctgtctagctccgagatgggctacacagccaccctgacaagaaccacaccaacattctttcccaaggacatcctgaccctgcggctggacgtgatgatggagacagagaaccgcctgcacttcaccatcaaggaccccgccaataggagatatgaggtgcctctggagaccccacacgtgcactctcgggcccctagcccactgtactccgtggagttctctgaggagccatttggcgtgatcgtgcggcgccagctggatggacgcgtgctgctgaacaccacagtggcccccctgttctttgccgaccagttcctccagctgagcacatccctgccctcccagtatatcaccggcctggccgagcacctgtctcctctgatgctgtctaccagctggacaaggatcaccctgtggaacagagacctggcaccaacccctggcgcaaatctgtacggcagccaccctttctatctggccctggaggatggaggctccgcccacggcgtgtttctgctgaactctaatgccatggacgtggtgctccagccaagccccgccctgtcctggcggtctaccggcggcatcctggacgtgtacatcttcctgggccctgagccaaagtccgtggtgcagcagtacctggacgtggtgggctatcctttcatgcccccttactggggactgggatttcacctgtgccgctggggctattctagcacagccatcacccggcaggtggtggagaacatgacccgcgcccactttccactggatgtgcagtggaatgacctggattacatggactccaggagagacttcaccttcaacaaggacggcttcagggattttcccgccatggtgcaggagctgcaccagggcggccggcgctacatgatgatcgtggaccccgccatctcctctagcggacctgccggcagctacagaccatatgacgagggcctgaggagaggcgtgttcatcacaaacgagaccggccagcctctgatcggcaaggtctggccaggctccaccgccttcccagacttcaccaatccaaccgccctggcctggtgggaggacatggtggccgagttccacgaccaggtgccttttgatggcatgtggatcgacatgaacgagccatctaatttcatcaggggcagcgaggacggctgccccaacaatgagctggagaacccaccatatgtgcctggcgtggtgggaggcaccctccaggcagcaaccatctgtgcctcctctcaccagtttctgtctacacactataacctgcacaatctgtacggactgaccgaggcaatcgccagccacagagccctggtgaaggccaggggcacaagacctttcgtgatctccaggtctacctttgccggacacggcagatacgcaggacactggaccggcgacgtgtggagcagctgggagcagctggcctctagcgtgccagagatcctccagttcaacctgctgggcgtgcccctggtgggagcagacgtgtgcggctttctgggcaatacatccgaggagctgtgcgtgaggtggacccagctgggagccttctatcccttcatgcgcaaccacaatagcctgctgtccctgcctcaggagccatacagcttctccgagcctgcacagcaggcaatgaggaaggccctgacactgcgctatgccctgctgccacacctgtacaccctgtttcaccaggcacacgtggcaggagagacagtggcccggcccctgttcctggagtttcctaaggattcctctacctggacagtggaccaccagctgctgtggggagaggccctgctgatcacccccgtgctccaggcaggcaaggcagaggtgacaggctatttccctctgggcacatggtacgacctccagaccgtgccagtggaggccctgggcagcctgcctccaccacctgccgccccccgcgagcctgccatccactccgagggacagtgggtgacactgccagcacctctggacaccatcaacgtgcacctgagggccggctatatcatccccctccagggccctggcctgaccacaaccgagtccagacagcagccaatggccctggccgtggccctgaccaagggaggcgaggccaggggcgagctgttctgggacgatggcgagtctctggaggtgctggagagaggcgcctacacacaggtcatcttcctggccaggaacaatacaatcgtgaatgagctggtgagagtgacctctgagggagcaggactccagctccagaaggtgacagtgctgggagtggcaaccgcaccacagcaggtgctgagcaacggcgtgcccgtgagcaatttcacatactcccctgataccaaggtgctggacatctgcgtgagcctgctgatgggcgagcagtttctggtgtcctggtgttga

SEQ ID NO: 10 - DNA, 8523 bp, Artificial Sequence
  Dual promoter lentiviral vector
aaattgtaagcgttaatattttgttaaaattcgcgttaaatttttgttaaatcagctcattttttaaccaataggccgaaatcggcaaaatcccttataaatcaaaagaatagaccgagatagggttgagtgttgttccagtttggaacaagagtccactattaaagaacgtggactccaacgtcaaagggcgaaaaaccgtctatcagggcgatggcccactacgtgaaccatcaccctaatcaagttttttggggtcgaggtgccgtaaagcactaaatcggaaccctaaagggagcccccgatttagagcttgacggggaaagccggcgaacgtggcgagaaaggaagggaagaaagcgaaaggagcgggcgctagggcgctggcaagtgtagcggtcacgctgcgcgtaaccaccacacccgccgcgcttaatgcgccgctacagggcgcgtccattcgccattcaggctgcgcaactgttgggaagggcgatcggtgcgggcctcttcgctattacgccagctggcgaaagggggatgtgctgcaaggcgattaagttgggtaacgccagggttttcccagtcacgacgttgtaaaacgacggccagtgaattgtaatacgactcactatagggcgaattgggcccgacgtcgcatgcttggaagggctaattcactcccaaagaagacaagatatccttgatctgtggatctaccacacacaaggctacttccctgattagcagaactacacaccagggccaggggtcagatatccactgacctttggatggtgctacaagctagtaccagttgagccagataaggtagaagaggccaataaaggagagaacaccagcttgttacaccctgtgagcctgcatgggatggatgacccggagagagaagtgttagagtggaggtttgacagccgcctagcatttcatcacgtggcccgagagctgcatccggagtacttcaagaactgctgatatcgagcttgctacaagggactttccgctggggactttccagggaggcgtggcctgggcgggactggggagtggcgagccctcagatcctgcatataagcagctgctttttgcctgtactgggtctctctggttagaccagatctgagcctgggagctctctggctaactagggaacccactgcttaagcctcaataaagcttgccttgagtgcttcaagtagtgtgtgcccgtctgttgtgtgactctggtaactagagatccctcagacccttttagtcagtgtggaaaatctctagcagtggcgcccgaacagggacttgaaagcgaaagggaaaccagaggagctctctcgacgcaggactcggcttgctgaagcgcgcacggcaagaggcgaggggcggcgactggtgagtacgccaaaaattttgactagcggaggctagaaggagagagatgggtgcgagagcgtcagtattaagcgggggagaattagatcgcgatgggaaaaaattcggttaaggccagggggaaagaaaaaatataaattaaaacatatagtatgggcaagcagggagctagaacgattcgcagttaatcctggcctgttagaaacatcagaaggctgtagacaaatactgggacagctacaaccatcccttcagacaggatcagaagaacttagatcattatataatacagtagcaaccctctattgtgtgcatcaaaggatagagataaaagacaccaaggaagctttagacaagatagaggaagagcaaaacaaaagtaagaccaccgcacagcaagcggccgctgatcttcagacctggaggaggagatatgagggacaattggagaagtgaattatataaatataaagtagtaaaaattgaaccattaggagtagcacccaccaaggcaaagagaagagtggtgcagagagaaaaaagagcagtgggaataggagctttgttccttgggttcttgggagcagcaggaagcactatgggcgcagcgtcaatgacgctgacggtacaggccagacaattattgtctggtatagtgcagcagcagaacaatttgctgagggctattgaggcgcaacagcatctgttgcaactcacagtctggggcatcaagcagctccaggcaagaatcctggctgtggaaagatacctaaaggatcaacagctcctggggatttggggttgctctggaaaactcatttgcaccactgctgtgccttggaatgctagttggagtaataaatctctggaacagatttggaatcacacgacctggatggagtgggacagagaaattaacaattacacaagcttaatacactccttaattgaagaatcgcaaaaccagcaagaaaagaatgaacaagaattattggaattagataaatgggcaagtttgtggaattggtttaacataacaaattggctgtggtatataaaattattcataatgatagtaggaggcttggtaggtttaagaatagtttttgctgtactttctatagtgaatagagttaggcagggatattcaccattatcgtttcagacccacctcccaaccccgaggggacccgacaggcccgaaggaatagaagaagaaggtggagagagagacagagacagatccattcgattagtgaacggatctcgacgggatcgattttaaaagaaaaggggggattggggggtacagtgcaggggaaagaatagtagacataatagcaacagacatacaaactaaagaattacaaaaacaaattacaaaaattcaaaattttatcgataagctttgcaaagatggataaagttttaaacagagaggaatctttgcagctaatggaccttctaggtctgaccccgtacgcctcgagagatctgatcataatcagccataccacatttgtagaggttttacttgctttaaaaaacctcccacacctccccctgaacctgaaacataaaatgaatgcaattgttgttgttaacttgtttattgcagcttataatggttacaaataaggcaatagcatcacaaatttcacaaataaggcatttttttcactgcattctagttttggtttgtccaaactcatcaatgtatcttatcatgtctggatctcaaatccctcggaagctgcgcctgtcttaggttggagtgatacatttttatcacttttacccgtctttggattaggcagtagctctgacggccctcctgtcttaggttagtgaaaaatgtcactctcttacccgtcattggctgtccagcttagctcgcaggggaggtggtctgcctgcaggcggatggcgttaacatatgacaactttctcccgggtaatctgaccgttcgctagccctggggagagaggtcggtgattcggtcaacgagggagccgactgccgacgtgcgctccggaggcttgcagaatgcggaacaccgcgcgggcaggaacagggcccacactaccgccccacaccccgcctcccgcaccgccccttcccggccgctgctctcggcgcgccccgctgagcagccgctattggccacagcccatcgcggtcggcgcgctgccattgctccctggcgctgtccgtctgcgagggtactagtgagacgtgcggcttccgtttgtcacgtccggcacgccgcgaaccgcaaggaaccttcccgacttaggggcggagcaggaagcgtcgccggggggcccacaagggtagcggcgaagatccgggtgacgctgcgaacggacgtgaagaatgtgcgagacccagggtcggcgccgctgcgtttcccggaaccacgcccagagcagccgcgtccctgcgcaaacccagggctgccaaggaaaaggcgcaaccccaaccccgtggttaattaaggtgaaaggagtgggaattggctccggtgcccgtcagtgggcagagcgcacatcgcccacagtccccgagaagttggggggaggggtcggcaattgaaccggtgcctagagaaggtggcgcggggtaaactgggaaagtgatgtcgtgtactggctccgcctttttcccgagggtgggggagaaccgtatataagtgcagtagtcgccgtgaacgttctttttcgcaacgggtttgccgccagaacacaggtaagtgccgtgtgtggttcccgcgggcctggcctctttacgggttatggcccttgcgtgccttgaattacttccacctggctgcagtacgtgattcttgatcccgagcttcgggttggaagtgggtgggagagttcgaggccttgcgcttaaggagccccttcgcctcgtgcttgagttgaggcctggcctgggcgctggggccgccgcgtgcgaatctggtggcaccttcgcgcctgtctcgctgctttcgataagtctctagccatttaaaatttttgatgacctgctgcgacgctttttttctggcaagatagtcttgtaaatgcgggccaagatctgcacactggtatttcggtttttggggccgcgggcggcgacggggcccgtgcgtcccagcgcacatgttcggcgaggcggggcctgcgagcgcggccaccgagaatcggacgggggtagtctcaagctggccggcctgctctggtgcctggcctcgcgccgccgtgtatcgccccgccctgggcggcaaggctggcccggtcggcaccagttgcgtgagcggaaagatggccgcttcccggccctgctgcagggagctcaaaatggaggacgcggcgctcgggagagcgggcgggtgagtcacccacacaaaggaaaagggcctttccgtcctcagccgtcgcttcatgtgactccacggagtaccgggcgccgtccaggcacctcgattagttctcgagcttttggagtacgtcgtctttaggttggggggaggggttttatgcgatggagtttccccacactgagtgggtggagactgaagttaggccagcttggcacttgatgtaattctccttggaatttgccctttttgagtttggatcttggttcattctcaagcctcagacagtggttcaaagtttttttcttccatttcaggtgtcgtgaggaattctgcagtcgacggtaccgcgggcgcgccccgggatccaagcttcaattgtggtcactcgacaatcaacctctggattacaaaatttgtgaaagattgactggtattcttaactatgttgctccttttacgctatgtggatacgctgctttaatgcctttgtatcatgctattgcttcccgtatggctttcattttctcctccttgtataaatcctggttgctgtctctttatgaggagttgtggcccgttgtcaggcaacgtggcgtggtgtgcactgtgtttgctgacgcaacccccactggttggggcattgccaccacctgtcagctcctttccgggactttcgctttccccctccctattgccacggcggaactcatcgccgcctgccttgcccgctgctggacaggggctcggctgttgggcactgacaattccgtggtgttgtcggggaagctgacgtcctttccatggctgctcgcctgtgttgccacctggattctgcgcgggacgtccttctgctacgtcccttcggccctcaatccagcggaccttccttcccgcggcctgctgccggctctgcggcctcttccgcgtcttcgccttcgccctcagacgagtcggatctccctttgggccgcctccccgcctgctcgagacctagaaaaacatggagcaatcacaagtagcaatacagcagctaccaatgctgattgtgcctggctagaagcacaagaggaggaggaggtgggttttccagtcacacctcaggtacctttaagaccaatgacttacaaggcagctgtagatcttagccactttttaaaagaaaaggggggactggaagggctaattcactcccaacgaagacaagatctgctttttgcttgtactgggtctctctggttagaccagatctgagcctgggagctctctggctaactagggaacccactgcttaagcctcaataaagcttgccttgagtgcttcaagtagtgtgtgcccgtctgttgtgtgactctggtaactagagatccctcagacccttttagtcagtgtggaaaatctctagcagtagtagttcatgtcatcttattattcagtatttataacttgcaaagaaatgaatatcagagagtgagaggacgcgttggatgcatagcttgagtattctatagtgtcacctaaatagcttggcgtaatcatggtcatagctgtttcctgtgtgaaattgttatccgctcacaattccacacaacatacgagccggaagcataaagtgtaaagcctggggtgcctaatgagtgagctaactcacattaattgcgttgcgctcactgcccgctttccagtcgggaaacctgtcgtgccagctgcattaatgaatcggccaacgcgcggggagaggcggtttgcgtattgggcgctcttccgcttcctcgctcactgactcgctgcgctcggtcgttcggctgcggcgagcggtatcagctcactcaaaggcggtaatacggttatccacagaatcaggggataacgcaggaaagaacatgtgagcaaaaggccagcaaaaggccaggaaccgtaaaaaggccgcgttgctggcgtttttccataggctccgcccccctgacgagcatcacaaaaatcgacgctcaagtcagaggtggcgaaacccgacaggactataaagataccaggcgtttccccctggaagctccctcgtgcgctctcctgttccgaccctgccgcttaccggatacctgtccgcctttctcccttcgggaagcgtggcgctttctcatagctcacgctgtaggtatctcagttcggtgtaggtcgttcgctccaagctgggctgtgtgcacgaaccccccgttcagcccgaccgctgcgccttatccggtaactatcgtcttgagtccaacccggtaagacacgacttatcgccactggcagcagccactggtaacaggattagcagagcgaggtatgtaggcggtgctacagagttcttgaagtggtggcctaactacggctacactagaagaacagtatttggtatctgcgctctgctgaagccagttaccttcggaaaaagagttggtagctcttgatccggcaaacaaaccaccgctggtagcggtggtttttttgtttgcaagcagcagattacgcgcagaaaaaaaggatctcaagaagatcctttgatcttttctacggggtctgacgctcagtggaacgaaaactcacgttaagggattttggtcatgagattatcaaaaaggatcttcacctagatccttttaaattaaaaatgaagttttaaatcaatctaaagtatatatgagtaaacttggtctgacagttaccaatgcttaatcagtgaggcacctatctcagcgatctgtctatttcgttcatccatagttgcctgactccccgtcgtgtagataactacgatacgggagggcttaccatctggccccagtgctgcaatgataccgcgagacccacgctcaccggctccagatttatcagcaataaaccagccagccggaagggccgagcgcagaagtggtcctgcaactttatccgcctccatccagtctattaattgttgccgggaagctagagtaagtagttcgccagttaatagtttgcgcaacgttgttgccattgctacaggcatcgtggtgtcacgctcgtcgtttggtatggcttcattcagctccggttcccaacgatcaaggcgagttacatgatcccccatgttgtgcaaaaaagcggttagctccttcggtcctccgatcgttgtcagaagtaagttggccgcagtgttatcactcatggttatggcagcactgcataattctcttactgtcatgccatccgtaagatgcttttctgtgactggtgagtactcaaccaagtcattctgagaatagtgtatgcggcgaccgagttgctcttgcccggcgtcaatacgggataataccgcgccacatagcagaactttaaaagtgctcatcattggaaaacgttcttcggggcgaaaactctcaaggatcttaccgctgttgagatccagttcgatgtaacccactcgtgcacccaactgatcttcagcatcttttactttcaccagcgtttctgggtgagcaaaaacaggaaggcaaaatgccgcaaaaaagggaataagggcgacacggaaatgttgaatactcatactcttcctttttcaatattattgaagcatttatcagggttattgtctcatgagcggatacatatttgaatgtatttagaaaaataaacaaataggggttccgcgcacatttccccgaaaagtgccacctgatgcggtgtgaaataccgcacagatgcgtaaggagaaaataccgcatcagg

SEQ ID NO: 11 - DNA, 10025 bp, Artificial Sequence
  Dual promoter lentiviral vector comprising IMPDH2(IY) resistance gene
aaattgtaagcgttaatattttgttaaaattcgcgttaaatttttgttaaatcagctcattttttaaccaataggccgaaatcggcaaaatcccttataaatcaaaagaatagaccgagatagggttgagtgttgttccagtttggaacaagagtccactattaaagaacgtggactccaacgtcaaagggcgaaaaaccgtctatcagggcgatggcccactacgtgaaccatcaccctaatcaagttttttggggtcgaggtgccgtaaagcactaaatcggaaccctaaagggagcccccgatttagagcttgacggggaaagccggcgaacgtggcgagaaaggaagggaagaaagcgaaaggagcgggcgctagggcgctggcaagtgtagcggtcacgctgcgcgtaaccaccacacccgccgcgcttaatgcgccgctacagggcgcgtccattcgccattcaggctgcgcaactgttgggaagggcgatcggtgcgggcctcttcgctattacgccagctggcgaaagggggatgtgctgcaaggcgattaagttgggtaacgccagggttttcccagtcacgacgttgtaaaacgacggccagtgaattgtaatacgactcactatagggcgaattgggcccgacgtcgcatgcttggaagggctaattcactcccaaagaagacaagatatccttgatctgtggatctaccacacacaaggctacttccctgattagcagaactacacaccagggccaggggtcagatatccactgacctttggatggtgctacaagctagtaccagttgagccagataaggtagaagaggccaataaaggagagaacaccagcttgttacaccctgtgagcctgcatgggatggatgacccggagagagaagtgttagagtggaggtttgacagccgcctagcatttcatcacgtggcccgagagctgcatccggagtacttcaagaactgctgatatcgagcttgctacaagggactttccgctggggactttccagggaggcgtggcctgggcgggactggggagtggcgagccctcagatcctgcatataagcagctgctttttgcctgtactgggtctctctggttagaccagatctgagcctgggagctctctggctaactagggaacccactgcttaagcctcaataaagcttgccttgagtgcttcaagtagtgtgtgcccgtctgttgtgtgactctggtaactagagatccctcagacccttttagtcagtgtggaaaatctctagcagtggcgcccgaacagggacttgaaagcgaaagggaaaccagaggagctctctcgacgcaggactcggcttgctgaagcgcgcacggcaagaggcgaggggcggcgactggtgagtacgccaaaaattttgactagcggaggctagaaggagagagatgggtgcgagagcgtcagtattaagcgggggagaattagatcgcgatgggaaaaaattcggttaaggccagggggaaagaaaaaatataaattaaaacatatagtatgggcaagcagggagctagaacgattcgcagttaatcctggcctgttagaaacatcagaaggctgtagacaaatactgggacagctacaaccatcccttcagacaggatcagaagaacttagatcattatataatacagtagcaaccctctattgtgtgcatcaaaggatagagataaaagacaccaaggaagctttagacaagatagaggaagagcaaaacaaaagtaagaccaccgcacagcaagcggccgctgatcttcagacctggaggaggagatatgagggacaattggagaagtgaattatataaatataaagtagtaaaaattgaaccattaggagtagcacccaccaaggcaaagagaagagtggtgcagagagaaaaaagagcagtgggaataggagctttgttccttgggttcttgggagcagcaggaagcactatgggcgcagcgtcaatgacgctgacggtacaggccagacaattattgtctggtatagtgcagcagcagaacaatttgctgagggctattgaggcgcaacagcatctgttgcaactcacagtctggggcatcaagcagctccaggcaagaatcctggctgtggaaagatacctaaaggatcaacagctcctggggatttggggttgctctggaaaactcatttgcaccactgctgtgccttggaatgctagttggagtaataaatctctggaacagatttggaatcacacgacctggatggagtgggacagagaaattaacaattacacaagcttaatacactccttaattgaagaatcgcaaaaccagcaagaaaagaatgaacaagaattattggaattagataaatgggcaagtttgtggaattggtttaacataacaaattggctgtggtatataaaattattcataatgatagtaggaggcttggtaggtttaagaatagtttttgctgtactttctatagtgaatagagttaggcagggatattcaccattatcgtttcagacccacctcccaaccccgaggggacccgacaggcccgaaggaatagaagaagaaggtggagagagagacagagacagatccattcgattagtgaacggatctcgacgggatcgattttaaaagaaaaggggggattggggggtacagtgcaggggaaagaatagtagacataatagcaacagacatacaaactaaagaattacaaaaacaaattacaaaaattcaaaattttatcgataagctttgcaaagatggataaagttttaaacagagaggaatctttgcagctaatggaccttctaggtctgaccccgtacgcctcgagagatctgatcataatcagccataccacatttgtagaggttttacttgctttaaaaaacctcccacacctccccctgaacctgaaacataaaatgaatgcaattgttgttgttaacttgtttattgcagcttataatggttacaaataaggcaatagcatcacaaatttcacaaataaggcatttttttcactgcattctagttttggtttgtccaaactcatcaatgtatcttatcatgtctggatctcaaatccctcggaagctgcgcctgtcttaggttggagtgatacatttttatcacttttacccgtctttggattaggcagtagctctgacggccctcctgtcttaggttagtgaaaaatgtcactctcttacccgtcattggctgtccagcttagctcgcaggggaggtggtctgcctgcaggttagaacagtctcttttcgtatgagtgcagtgagtggacgccgccttcgacctgggctgaagaagttcttttctcgaacttcagttcgccggaatacatcattgcccgcacctgtgtcaggctcttagcgccgatatcctggcatgaatgctgaattccggcgatcaggtaaggcacgaatttgtgaatactgcccttatcctggacagctccagacacgccctgtgcgactttgatcttgtctgcctcggaaaaatacctgttctgagaggacagatgcttatccatggcgtccagtgaccccatgcccctatatttcttcagtctgaacccatcactaaagaagtactcgccgggggcttctgtggttgcagccagcaggctgcccatcatcactgtgcttgcccccagagccagggcttttgcgatgtggcccacattctgaattcccccgtcagcgatcactgggactccgaatctccgggcatactcgtacaccttgtagacagcagttgcctgaggtcgtccacaggccagcacttcctgaatgatgcagattgatccactccccattccgaccctcagagcatccactcctgcgtcaatcaggtttttggcctgggctgcggtcacgacattgcctccgatgacctgcagatttgggtacttgtccttaatgtacttgatcatattaatctggaagatgctgtttccctggcttgaatccagcacgaccacgtccacccctgcctgagccagcagatccaggcgatatttatcgtcctcgtgtgtgccaatagcggctccacacagcagctgtttctttgcgtccttactagccagagggtaatctcgatttttcttcaggtcggtgcgggcaatgattgccaccagctcatcgtcttcattcacgataggcagttttcctttcttagaccgctgcagaatctcgttggcttccttcagtgtgatgccggcaggtgcgaccaccagatcttcgcgtttggtcataatctcttccagaaaacagtcatgctcttcctccttcaggaaatcgatgtctcgactagaaatgattcccaccagtcggctgcccattcgtccagtatctgtaatggggatgccgcaaaatccgtgcctagctttggcctcgaacacatcgcggaccctgtccttggggctcaggaccactgggtcggtgataaagccctgttcgtatttcttcacctttctgacctcattggcctgaaattctggagtgcagttatggtgaatgaacccgatcccgcctgtcagtgccatagcaatggccatgccagcctcggtgacagtgtccataggggagctcaccaggggtgtcttcagggtgattttcttggtcagggcagaagtcagatccacctggtctgcggtaaaatcaatatagccgggcaggatcaggaagtcgttgtaagtcagcccgtctccacaattaaacagctgctgggcggtcagtccatcatcagggacataggaagtgcctccagaaatcaggtagtcggccatggtggcgctagccctggggagagaggtcggtgattcggtcaacgagggagccgactgccgacgtgcgctccggaggcttgcagaatgcggaacaccgcgcgggcaggaacagggcccacactaccgccccacaccccgcctcccgcaccgccccttcccggccgctgctctcggcgcgccccgctgagcagccgctattggccacagcccatcgcggtcggcgcgctgccattgctccctggcgctgtccgtctgcgagggtactagtgagacgtgcggcttccgtttgtcacgtccggcacgccgcgaaccgcaaggaaccttcccgacttaggggcggagcaggaagcgtcgccggggggcccacaagggtagcggcgaagatccgggtgacgctgcgaacggacgtgaagaatgtgcgagacccagggtcggcgccgctgcgtttcccggaaccacgcccagagcagccgcgtccctgcgcaaacccagggctgccaaggaaaaggcgcaaccccaaccccgtggttaattaaggtgaaaggagtgggaattggctccggtgcccgtcagtgggcagagcgcacatcgcccacagtccccgagaagttggggggaggggtcggcaattgaaccggtgcctagagaaggtggcgcggggtaaactgggaaagtgatgtcgtgtactggctccgcctttttcccgagggtgggggagaaccgtatataagtgcagtagtcgccgtgaacgttctttttcgcaacgggtttgccgccagaacacaggtaagtgccgtgtgtggttcccgcgggcctggcctctttacgggttatggcccttgcgtgccttgaattacttccacctggctgcagtacgtgattcttgatcccgagcttcgggttggaagtgggtgggagagttcgaggccttgcgcttaaggagccccttcgcctcgtgcttgagttgaggcctggcctgggcgctggggccgccgcgtgcgaatctggtggcaccttcgcgcctgtctcgctgctttcgataagtctctagccatttaaaatttttgatgacctgctgcgacgctttttttctggcaagatagtcttgtaaatgcgggccaagatctgcacactggtatttcggtttttggggccgcgggcggcgacggggcccgtgcgtcccagcgcacatgttcggcgaggcggggcctgcgagcgcggccaccgagaatcggacgggggtagtctcaagctggccggcctgctctggtgcctggcctcgcgccgccgtgtatcgccccgccctgggcggcaaggctggcccggtcggcaccagttgcgtgagcggaaagatggccgcttcccggccctgctgcagggagctcaaaatggaggacgcggcgctcgggagagcgggcgggtgagtcacccacacaaaggaaaagggcctttccgtcctcagccgtcgcttcatgtgactccacggagtaccgggcgccgtccaggcacctcgattagttctcgagcttttggagtacgtcgtctttaggttggggggaggggttttatgcgatggagtttccccacactgagtgggtggagactgaagttaggccagcttggcacttgatgtaattctccttggaatttgccctttttgagtttggatcttggttcattctcaagcctcagacagtggttcaaagtttttttcttccatttcaggtgtcgtgaggaattctgcagtcgacggtaccgcgggcgcgccccgggatccaagcttcaattgtggtcactcgacaatcaacctctggattacaaaatttgtgaaagattgactggtattcttaactatgttgctccttttacgctatgtggatacgctgctttaatgcctttgtatcatgctattgcttcccgtatggctttcattttctcctccttgtataaatcctggttgctgtctctttatgaggagttgtggcccgttgtcaggcaacgtggcgtggtgtgcactgtgtttgctgacgcaacccccactggttggggcattgccaccacctgtcagctcctttccgggactttcgctttccccctccctattgccacggcggaactcatcgccgcctgccttgcccgctgctggacaggggctcggctgttgggcactgacaattccgtggtgttgtcggggaagctgacgtcctttccatggctgctcgcctgtgttgccacctggattctgcgcgggacgtccttctgctacgtcccttcggccctcaatccagcggaccttccttcccgcggcctgctgccggctctgcggcctcttccgcgtcttcgccttcgccctcagacgagtcggatctccctttgggccgcctccccgcctgctcgagacctagaaaaacatggagcaatcacaagtagcaatacagcagctaccaatgctgattgtgcctggctagaagcacaagaggaggaggaggtgggttttccagtcacacctcaggtacctttaagaccaatgacttacaaggcagctgtagatcttagccactttttaaaagaaaaggggggactggaagggctaattcactcccaacgaagacaagatctgctttttgcttgtactgggtctctctggttagaccagatctgagcctgggagctctctggctaactagggaacccactgcttaagcctcaataaagcttgccttgagtgcttcaagtagtgtgtgcccgtctgttgtgtgactctggtaactagagatccctcagacccttttagtcagtgtggaaaatctctagcagtagtagttcatgtcatcttattattcagtatttataacttgcaaagaaatgaatatcagagagtgagaggacgcgttggatgcatagcttgagtattctatagtgtcacctaaatagcttggcgtaatcatggtcatagctgtttcctgtgtgaaattgttatccgctcacaattccacacaacatacgagccggaagcataaagtgtaaagcctggggtgcctaatgagtgagctaactcacattaattgcgttgcgctcactgcccgctttccagtcgggaaacctgtcgtgccagctgcattaatgaatcggccaacgcgcggggagaggcggtttgcgtattgggcgctcttccgcttcctcgctcactgactcgctgcgctcggtcgttcggctgcggcgagcggtatcagctcactcaaaggcggtaatacggttatccacagaatcaggggataacgcaggaaagaacatgtgagcaaaaggccagcaaaaggccaggaaccgtaaaaaggccgcgttgctggcgtttttccataggctccgcccccctgacgagcatcacaaaaatcgacgctcaagtcagaggtggcgaaacccgacaggactataaagataccaggcgtttccccctggaagctccctcgtgcgctctcctgttccgaccctgccgcttaccggatacctgtccgcctttctcccttcgggaagcgtggcgctttctcatagctcacgctgtaggtatctcagttcggtgtaggtcgttcgctccaagctgggctgtgtgcacgaaccccccgttcagcccgaccgctgcgccttatccggtaactatcgtcttgagtccaacccggtaagacacgacttatcgccactggcagcagccactggtaacaggattagcagagcgaggtatgtaggcggtgctacagagttcttgaagtggtggcctaactacggctacactagaagaacagtatttggtatctgcgctctgctgaagccagttaccttcggaaaaagagttggtagctcttgatccggcaaacaaaccaccgctggtagcggtggtttttttgtttgcaagcagcagattacgcgcagaaaaaaaggatctcaagaagatcctttgatcttttctacggggtctgacgctcagtggaacgaaaactcacgttaagggattttggtcatgagattatcaaaaaggatcttcacctagatccttttaaattaaaaatgaagttttaaatcaatctaaagtatatatgagtaaacttggtctgacagttaccaatgcttaatcagtgaggcacctatctcagcgatctgtctatttcgttcatccatagttgcctgactccccgtcgtgtagataactacgatacgggagggcttaccatctggccccagtgctgcaatgataccgcgagacccacgctcaccggctccagatttatcagcaataaaccagccagccggaagggccgagcgcagaagtggtcctgcaactttatccgcctccatccagtctattaattgttgccgggaagctagagtaagtagttcgccagttaatagtttgcgcaacgttgttgccattgctacaggcatcgtggtgtcacgctcgtcgtttggtatggcttcattcagctccggttcccaacgatcaaggcgagttacatgatcccccatgttgtgcaaaaaagcggttagctccttcggtcctccgatcgttgtcagaagtaagttggccgcagtgttatcactcatggttatggcagcactgcataattctcttactgtcatgccatccgtaagatgcttttctgtgactggtgagtactcaaccaagtcattctgagaatagtgtatgcggcgaccgagttgctcttgcccggcgtcaatacgggataataccgcgccacatagcagaactttaaaagtgctcatcattggaaaacgttcttcggggcgaaaactctcaaggatcttaccgctgttgagatccagttcgatgtaacccactcgtgcacccaactgatcttcagcatcttttactttcaccagcgtttctgggtgagcaaaaacaggaaggcaaaatgccgcaaaaaagggaataagggcgacacggaaatgttgaatactcatactcttcctttttcaatattattgaagcatttatcagggttattgtctcatgagcggatacatatttgaatgtatttagaaaaataaacaaataggggttccgcgcacatttccccgaaaagtgccacctgatgcggtgtgaaataccgcacagatgcgtaaggagaaaataccgcatcagg